European Patent Application EP 4 253 549 A2, published October 4, 2023. Title: IMPROVED HIGH-THROUGHPUT COMBINATORIAL GENETIC MODIFICATION SYSTEM AND OPTIMIZED CAS9 ENZYME VARIANTS. Applicant: THE UNIVERSITY OF HONG KONG. Application EP. The sequence listing filed with the application follows.

SEQUENCE LISTING (264 sequences)

SEQ ID NO: 1 - protein, 1368 aa, Streptococcus pyogenes [sequence omitted]

SEQ ID NO: 2 - DNA, 4647 bp, Streptococcus pyogenes
  source 1..4647: mol_type = unassigned DNA
atggccccaaagaagaagcggaaggtcggtatccacggagtcccagcagccgacaagaagtacagcatcggcctggacatcggcaccaactctgtgggctgggccgtgatcaccgacgagtacaaggtgcccagcaagaaattcaaggtgctgggcaacaccgaccggcacagcatcaagaagaacctgatcggagccctgctgttcgacagcggcgaaacagccgaggccacccggctgaagagaaccgccagaagaagatacaccagacggaagaaccggatctgctatctgcaagagatcttcagcaacgagatggccaaggtggacgacagcttcttccacagactggaagagtccttcctggtggaagaggataagaagcacgagcggcaccccatcttcggcaacatcgtggacgaggtggcctaccacgagaagtaccccaccatctaccacctgagaaagaaactggtggacagcaccgacaaggccgacctgcggctgatctatctggccctggcccacatgatcaagttccggggccacttcctgatcgagggcgacctgaaccccgacaacagcgacgtggacaagctgttcatccagctggtgcagacctacaaccagctgttcgaggaaaaccccatcaacgccagcggcgtggacgccaaggccatcctgtctgccagactgagcaagagcagacggctggaaaatctgatcgcccagctgcccggcgagaagaagaatggcctgttcggaaacctgattgccctgagcctgggcctgacccccaacttcaagagcaacttcgacctggccgaggatgccaaactgcagctgagcaaggacacctacgacgacgacctggacaacctgctggcccagatcggcgaccagtacgccgacctgtttctggccgccaagaacctgtccgacgccatcctgctgagcgacatcctgagagtgaacaccgagatcaccaaggcccccctgagcgcctctatgatcaagagatacgacgagcaccaccaggacctgaccctgctgaaagctctcgtgcggcagcagctgcctgagaagtacaaagagattttcttcgaccagagcaagaacggctacgccggctacattgacggcggagccagccaggaagagttctacaagttcatcaagcccatcctggaaaagatggacggcaccgaggaactgctcgtgaagctgaacagagaggacctgctgcggaagcagcggaccttcgacaacggcagcatcccccaccagatccacctgggagagctgcacgccattctgcggcggcaggaagatttttacccattcctgaaggacaaccgggaaaagatcgagaagatcctgaccttccgcatcccctactacgtgggccctctggccaggggaaacagcagattcgcctggatgaccagaaagagcgaggaaaccatcaccccctggaacttcgaggaagtggtggacaagggcgcttccgcccagagcttcatcgagcggatgaccaacttcgataagaacctgcccaacgagaaggtgctgcccaagcacagcctgctgtacgagtacttcaccgtgtataacgagctgaccaaagtgaaatacgtgaccgagggaatgagaaagcccgccttcctgagcggcgagcagaaaaaggccatcgtggacctgctgttcaagaccaaccggaaagtgaccgtgaagcagctgaaagaggactacttcaagaaaatcgagtgcttcgactccgtggaaatctccggcgtggaagatcggttcaacgcctccctgggcacataccacgatctgctgaaaattatcaaggacaaggacttcctggacaatgaggaaaacgaggacattctggaagatatcgtgctgaccctgacactgtttgaggacagagagatgatcgaggaacggctgaaaacctatgcccacctgttcgacgacaaagtgatgaagcagctgaagcggcggagatacaccggctggggcaggctgagccggaagctgatcaacggcatccgggacaagcagtccggcaagacaatcctggatttcctgaagtccgacggcttcgccaacagaaacttcatgcagctgatccacgacgacagcctgacctttaaagaggacatccagaaagcccaggtgtccggccagggcgatagcctgcacgagcacattgccaatctggccggcagccccgccattaagaagggcatcctgcagacagtgaaggtggtggacgagctcgtgaaagtgatgggccggcacaagcccgagaacatcgtgatcgaaatggccagagagaaccagaccacccagaagggacagaagaacagccgcgagagaatgaagcggatcgaagagggcatcaaagagctgggcagccagatcctgaaagaacaccccgtggaaaacacccagctgcagaacgagaagctgtacctgtactacctgcagaatgggcgggatatgtacgtggaccaggaactggacatcaaccggctgtccgactacgatgtggaccatatcgtgcctcagagctttctgaaggacgactccatcgacaacaaggtgctgaccagaagcgacaagaaccggggcaagagcgacaacgtgccctccgaagaggtcgtgaagaagatgaagaactactggcggcagctgctgaacgccaagctgattacccagagaaagttcgacaatctgaccaaggccgagagaggcggcctgagcgaactggataaggccggcttcatcaagagacagctggtggaaacccggcagatcacaaagcacgtggcacagatcctggactcccggatgaacactaagtacgacgagaatgacaagctgatccgggaagtgaaagtgatcaccctgaagtccaagctggtgtccgatttccggaaggatttccagttttacaaagtgcgcgagatcaacaactaccaccacgcccacgacgcctacctgaacgccgtcgtgggaaccgccctgatcaaaaagtaccctaagctggaaagcgagttcgtgtacggcgactacaaggtgtacgacgtgcggaagatgatcgccaagagcgagcaggaaatcggcaaggctaccgccaagtacttcttctacagcaacatcatgaactttttcaagaccgagattaccctggccaacggcgagatccggaagcggcctctgatcgagacaaacggcgaaaccggggagatcgtgtgggataagggccgggattttgccaccgtgcggaaagtgctgagcatgccccaagtgaatatcgtgaaaaagaccgaggtgcagacaggcggcttcagcaaagagtctatcctgcccaagaggaacagcgataagctgatcgccagaaagaaggactgggaccctaagaagtacggcggcttcgacagccccaccgtggcctattctgtgctggtggtggccaaagtggaaaagggcaagtccaagaaactgaagagtgtgaaagagctgctggggatcaccatcatggaaagaagcagcttcgagaagaatcccatcgactttctggaagccaagggctacaaagaagtgaaaaaggacctgatcatcaagctgcctaagtactccctgttcgagctggaaaacggccggaagagaatgctggcctctgccggcgaactgcagaagggaaacgaactggccctgccctccaaatatgtgaacttcctgtacctggccagccactatgagaagctgaagggctcccccgaggataatgagcagaaacagctgtttgtggaacagcacaagcactacctggacgagatcatcgagcagatcagcgagttctccaagagagtgatcctggccgacgctaatctggacaaagtgctgtccgcctacaacaagcaccgggataagcccatcagagagcaggccgagaatatcatccacctgtttaccctgaccaatctgggagcccctgccgccttcaagtactttgacaccaccatcgaccggaagaggtacaccagcaccaaagaggtgctggacgccaccctgatccaccagagcatcaccggcctgtacgagacacggatcgacctgtctcagctgggaggcgacaagcgtcctgctgctactaagaaagctggtcaagctaagaaaaagaaagctagcggcagcggcgccaccaacttcagcctgctgaagcaggccggcgacgtggaggagaaccccggccccatggccaagttgaccagtgccgttccggtgctcaccgcgcgcgacgtcgccggagcggtcgagttctggaccgaccggctcgggttctcccgggacttcgtggaggacgacttcgccggtgtggtccgggacgacgtgaccctgttcatcagcgcggtccaggaccaggtggtgccggacaacaccctggcctgggtgtgggtgcgcggcctggacgagctgtacgccgagtggtcggaggtcgtgtccacgaacttccgggacgcctccgggccggccatgaccgagatcggcgagcagccgtgggggcgggagttcgccctgcgcgacccggccggcaactgcgtgcacttcgtggccgaggagcaggactga

SEQ ID NO: 3 - protein, 1368 aa, synthetic construct
  REGION 1..1368: note = base sequence SEQ ID NO: 1, residue 1003 substituted with Histidine and residue 661 substituted with Alanine
MDKKYSIGLDIGTNSVGWAVITDEYKVPSKKFKVLGNTDRHSIKKNLIGALLFDSGETAEATRLKRTARRRYTRRKNRICYLQEIFSNEMAKVDDSFFHRLEESFLVEEDKKHERHPIFGNIVDEVAYHEKYPTIYHLRKKLVDSTDKADLRLIYLALAHMIKFRGHFLIEGDLNPDNSDVDKLFIQLVQTYNQLFEENPINASGVDAKAILSARLSKSRRLENLIAQLPGEKKNGLFGNLIALSLGLTPNFKSNFDLAEDAKLQLSKDTYDDDLDNLLAQIGDQYADLFLAAKNLSDAILLSDILRVNTEITKAPLSASMIKRYDEHHQDLTLLKALVRQQLPEKYKEIFFDQSKNGYAGYIDGGASQEEFYKFIKPILEKMDGTEELLVKLNREDLLRKQRTFDNGSIPHQIHLGELHAILRRQEDFYPFLKDNREKIEKILTFRIPYYVGPLARGNSRFAWMTRKSEETITPWNFEEVVDKGASAQSFIERMTNFDKNLPNEKVLPKHSLLYEYFTVYNELTKVKYVTEGMRKPAFLSGEQKKAIVDLLFKTNRKVTVKQLKEDYFKKIECFDSVEISGVEDRFNASLGTYHDLLKIIKDKDFLDNEENEDILEDIVLTLTLFEDREMIEERLKTYAHLFDDKVMKQLKRRRYTGWGALSRKLINGIRDKQSGKTILDFLKSDGFANRNFMQLIHDDSLTFKEDIQKAQVSGQGDSLHEHIANLAGSPAIKKGILQTVKVVDELVKVMGRHKPENIVIEMARENQTTQKGQKNSRERMKRIEEGIKELGSQILKEHPVENTQLQNEKLYLYYLQNGRDMYVDQELDINRLSDYDVDHIVPQSFLKDDSIDNKVLTRSDKNRGKSDNVPSEEVVKKMKNYWRQLLNAKLITQRKFDNLTKAERGGLSELDKAGFIKRQLVETRQITKHVAQILDSRMNTKYDENDKLIREVKVITLKSKLVSDFRKDFQFYKVREINNYHHAHDAYLNAVVGTALIKKYPHLESEFVYGDYKVYDVRKMIAKSEQEIGKATAKYFFYSNIMNFFKTEITLANGEIRKRPLIETNGETGEIVWDKGRDFATVRKVLSMPQVNIVKKTEVQTGGFSKESILPKRNSDKLIARKKDWDPKKYGGFDSPTVAYSVLVVAKVEKGKSKKLKSVKELLGITIMERSSFEKNPIDFLEAKGYKEVKKDLIIKLPKYSLFELENGRKRMLASAGELQKGNELALPSKYVNFLYLASHYEKLKGSPEDNEQKQLFVEQHKHYLDEIIEQISEFSKRVILADANLDKVLSAYNKHRDKPIREQAENIIHLFTLTNLGAPAAFKYFDTTIDRKRYTSTKEVLDATLIHQSITGLYETRIDLSQLGGD

SEQ ID NO: 4 - protein, 1345 aa, Streptococcus mutans
MKKPYSIGLDIGTNSVGWAVVTDDYKVPAKKMKVLGNTDKSHIKKNLLGALLFDSGNTAEDRRLKRTARRRYTRRRNRILYLQEIFSEEMGKVDDSFFHRLDESFLTDDDKNFDSHPIFGNKAEEDAYHQKFPTIYHLRKHLADSTEKADLRLVYLALAHMIKFRGHFLIEGELNAENTDVQKLFADFVGVYDRTFDDSHLSEITVDASSILTEKISKSRRLEKLINNYPKEKKNTLFGNLIALSLGLQPNFKTNFKLSEDAKLQFSKDTYEEELEVLLAQIGDNYAELFLSAKKLYDSILLSGILTVTDVSTKAPLSASMIQRYNEHQMDLAQLKQFIRQKLSDKYNEVFSDVSKDGYAGYIDGKTNQEAFYKYLKGLLNKIEGSGYFLDKIEREDFLRKQRTFDNGSIPHQIHLQEMRAIIRRQAEFYPFLADNQDRIEKILTFRIPYYVGPLARGKSDFAWLSRKSADKITPWNFDEIVDKESSVEAFINRMTNYDLYLPNQKVLPKHSLLYEKFTVYNELTKVKYKTEQGKTAFFDANMKQEIFDGVFKVYRKVTKDKLMDFLEKEFDEFRIVDLTGLDKENKAFNASYGTYHDLRKILDKDFLDNSKNEKILEDIVLTLTLFEDREMIRKRLKNYSDLLTKEQLKKLERRHYTGWGRLSAELIHGIRNKESRKTILDYLIDDGNSNRNFMQLINDDALSFKEEIAKAQVIGETDNLNQVVSDIAGSPAIKKGILQSLKIVDELVKIMGHQPENIVVEMARENQFTNQGRRNSQQRLKGLTDSIKEFGSQILKEHPVENSQLQNDRLFLYYLQNGRDMYTGEELDIDYLSQYDIDHIIPQAFIKDNSIDNRVLTSSKENRGKSDDVPSKDVVRKMKSYWSKLLSAKLITQRKFDNLTKGERGGLTDDDKAGFIKRQLVETRQITKHVARILDERFNTETDENNKKIRQVKIVTLKSNLVSNFRKEFELYKVREINDYHHAHDAYLNAVIGKALLGVYPQLEPEFVYGDYPHFHGHKENKATAKKFFYSNIMNFFKKDDVRTDKNGEIIWKKDEYISNIKKVLSYPQVNIVKKVEEQTGGFSKESILPKGDSDKLIPRKTKKFYWDTKKYGGFDSPIVAYSILVIADIEKGKSKKLKTVKALVGVTIMEKMTFERDPVAFLERKGYRNVQEENIIKLPKYSLFKLENGRKRLLASARELQKGNEIVLPNHLGTLLYHAKNIHKVDEPKHLDYVDKHKDEFKELLDVVSNFSKKYTLAEGNLEKIKELYAQNNGEDLKELASSFINLLTFTAIGAPATFKFFDKNIDRKRYTSTTEILNATLIHQSITGLYETRIDLSKLGGD

SEQ ID NO: 5 - protein, 1371 aa, Streptococcus dysgalactiae
MDKKYSIGLDIGTNSVGWAVITDDYKVPSKKFKVLGNTDRHSIKKNLIGALLFDSGETAEATRLKRTARRRYTRRKNRIRYLQEIFSSEMSKVDDSFFHRLEESFLVEEDKKHERHPIFGNIVDEVAYHEKYPTIYHLRKKLADSTDKADLRLIYLALAHMIKFRGHFLIEGDLNPDNSDMDKLFIQLVQTYNQLFEENPINASRVDAKAILSARLSKSRRLENLIAQLPGEKRNGLFGNLIALSLGLTPNFKSNFDLAEDAKLQLSKDTYDDDLDNLLAQIGDQYADLFLAAKNLSDAILLSDILRVNSEITKAPLSASMIKRYDEHHQDLTLLKALVRQQLPEKYKEIFFDQSKNGYAGYIDGGASQEEFYKFIKPILEKMDGTEELLAKLNREDLLRKQRTFDNGSIPHQIHLGELHAILRRQEDFYPFLKDNREKIEKILTFRIPYYVGPLARGNSRFAWMTRKSEETITPWNFEEVVDKGASAQSFIERMTNFDKNLPNEKVLPKHSLLYEYFTVYNELTKVKYVTEGMRKPAFLSGEQKKAIVDLLFKTNRKVTVKQLKEDYFKKIECFDSVEISGVEDRFNASLGTYHDLLKIIKDKDFLDNEENEDILEDIVLTLTLFEDKEMIEERLKKYANLFDDKVMKQLKRRHYTGWGRLSRKLINGIRDKQSGKTILDFLKSDGFANRNFMQLINDDSLTFKEAIQKAQVSGQGHSLHEQIANLAGSPAIKKGILQSVKVVDELVKVMGHKPENIVIEMARENQTTQKGQKNSRERMKRIEEGIKELGSQILKEHPVENTQLQNEKLYLYYLQNGRDMYVDQELDINRLSDYDVDHIVPQSFIKDDSIDNKVLTRSDKNRGKSDNVPSEEVVKKMKNYWRQLLNAKLITQRKFDNLTKAERGGLSELDKAGFIKRQLVETRQITKHVAQILDSRMNTKYDENDKLIREVKVITLKSKLVSDFRKDFQFYKVREINNYHHAHDAYLNAVVGTALIKKYPKLESEFVYGDYKVYDVRKMIAKSEQEIGKATAKRFFYSNIMNFFKTEITLANGEIRKRPLIETNEETGEIVWDKGRDFATVRKVLSMPQVNIVKKTEVQTGALTNESIYARGSFDKLISRKHRFESSKYGGFGSPTVTYSVLVVAKSKVQDGKVKKIKTGKELIGITLLDKLVFEKNPLKFIEDKGYGNVQIDKCIKLPKYSLFEFENGTRRMLASVMANNNSRGDLQKANEMFLPAKLVTLLYHAHKIESSKELEHEAYILDHYNDLYQLLSYIERFASLYVDVEKNISKVKELFSNIESYSISEICSSVINLLTLTASGAPADFKFLGTTIPRKRYGSPQSILSSTLIHQSITGLYETRIDLSQLGGD

SEQ ID NO: 6 - protein, 1348 aa, Streptococcus equi
MKKPYTIALDIGTNSVGWVVVTDDYRVPTKKMKVLGNTERKTIKKNLIGALLFDSGDTAEGTRLKRTARPRYTRRKNRLRFLKEIFTEEMAKVDDGFFQRLEDSFYVLEDKEGNKHPIFANLADEVAYHKKYPTIYHLRKELVDNPQKADLRLIYLAVAHIIKFRGHFLIEGTLSSKNNNLQKSFDHLVDTYNLLFEEQRLLTEGINAKELLSAALSKSKRLENLISLIPGQKKTGIFGNIIALSLGLTPNFKANFGLSKDVKLQLAKDTYADDLDSLLAQIGDQYADLFLAAKNLSDAILLSDILTESDEITRAPLSASMVKRYREHHKDLVTLKTLIKDQLPEKYQEIFLDKTKNGYAGYIEGQVSQEEFYKYLKPILARLDGSEPLLLKIDREDFLRKQRTFDNGSIPHQIHLEELHAILRRQEVFYPFLKDNRKKIESLLTFRIPYYVGPLARGHSRFAWVKRKFDGAIRPWNFEEIVDEEASAQIFIEKMTKNDLYLPNEKVLPKHSLLYETFTVYNELTKVKYATEGMTRPQFLSADQKQAIVDLLFKTNRKVTVKQLKENYFKKIECWDSVEITGVEDSFNASLGTYHDLLKIIQDKDFLDNPDNQKIIEDIILTLTLFEDKKMISKRLDQYAHLFDKVVLNKLERHHYTGWGRLSGKLINGIRDKQSGKTILDFLKADGFANRNFMQLIHDSELSFIDEIAKAQVIGKTEYSKDLVGNLAGSPAIKKGISQTIKIVDELVKIMGYLPQQIVIEMARENQTTAQGIKNARQRMRKLEETAKKLGSNILKEHPVDNSQLQNDKRYLYYLQNGKDMYTGDDLDIDYLSSYDIDHIIPQSFIKNNSIDNKVLTSQGANRGKLDNVPSEAIVRKMKGYWQSLLRAGAISKQKFDNLTKAERGGLTQVDKAGFIQLQLVETRQITKHVAQILDSRFNTEFDDHNKRIRKVHIITLKSKLVSDFRKEFGLYKIRDINHYHHAHDAYLNAVVAKAILGKYPQLAPEFVYGDYPKYNSFKERQKATQKTLFYSNILKFFKDQESLHVNSDGEEIWNANKHLPIIKNVLSIPQVNIVKKTEVQTGGFYKESILSKGNSDKLIPRKNNWDTRKYGGFDSPTVAYSVLVIAKMEKGKAKVLKPVKEMVGITIMERIAFEENPVVFLEAKGYREIQEHLIIKLPKYSLFELENGRRRLLASASELQKGNELFLPVDYMTFLYLAAHYHELTGSSEDVLRKKYFVERHLHYFDDIIQMINDFAERHILASSNLEKINHTYHNNSDLPVNERAENIINVFTFVALGAPAAFKFFDATIDRKRYTSTKEVLNATLIHQSVTGLYETRIDLSQLGEN

SEQ ID NO: 7 - protein, 1376 aa, Streptococcus oralis
MNNKPYSIGLDIGTNSVGWAVITDDYKVPSKKMKVLGNTDKHFIKKNLLGALLFDEGTTAEDRRLKRTARRRYTRRKNRLRYLQEIFTEEMSKVDSNFFHRLDDSFLVPEDKRGSKYPIFATLEEEKEYHKNFPTIYHLRKHLADSKEKADFRLIYLALAHMIKYRGHFLYEESFDIKNNDIQKIFNEFISIYDNTFEGSSLNGQNAQVEAIFTDKISKSAKRERVLKLFPDEKSTGLFSEFLKLIVGNQADFKKHFDLEEKAPLQFSKDTYDEDLENLLGQIGDDFADLFLVAKKLYDAILLSGILTVTDPSTKAPLSASMIERYENHQKDLATLKQFIKNNLPEKYDEVFSDQSKDGYAGYIDGKTTQEAFYKYIKNLLSKLEGADYFLDKIEREDFLRKQRTFDNGSIPHQIHLQEMNAIIRRQGEHYPFLQENKEKIEKILTFRIPYYVGPLARGNRDFAWLTRNSDQAIRPWNFEEVVDKARSAEDFINKMTNYDLYLPEEKVLPKHSLLYETFAVYNELTKVKFIAEGLRDYQFLDSGQKKQIVTQLFKEKRKVTEKDIIQYLHTVDGYDGIELKGIEKQFNASLSTYHDLLKIIKDKEFMDDSKNEAILENIVHTLTIFEDREMIRQHLTQYASIFDEKVIKALTRRHYTGWGKLSAKLINGICDKQTGDTILDYLIDDGEINRNFMQLIHDDGLSFKEIIQKAQVVGKTDDVKQVVQELPGSPAIKKGILQSIKIVDELVKVMGHEPESIVIEMARENQTTARGKKNSQQRYKRIEDALKNLAPELDSNILKEHPTDNIQLQNDRLFLYYLQNGKDMYTGEALDINQLSSCDIDHIIPQAFIKDDSLDNRVLTSSKDNRGKSDNVPSLEIVQKRKAFWQQLLDSKLISERKFNNLTKAERGGLDERDKVGFIRRQLVETRQITKHVAQILDARFNTEVTEKDKKDRSVKIITLKSNLVSNFRKEFRLYKVREINDYHHAHDAYLNAVVAKAILKKYPKLEPEFVYGDYQKYDLKRYISRTKDPKEVEKATEKYFFYSNLLNFFKEEVHYADGTIVKRENIEYSKDTGEIAWNKEKDFATIKKVLSLPQVNIVKKTEEQTVGQNGGLFDNNIVSKKKVVDASKLTPIKSGLSPEKYGGYARPTIAYSVLVIADIEKGKAKKLKRIKEMVGITVQDKKKFEANPIAYLEECGYKNINPNLIIKLPKYSLFEFNNGQRRLLASSIELQKGNELIVPYHFTALLYHAQRINKISEPIHKQYVETHQSEFKELLTAIISLSKKYIQKPNVESLLQQAFDQSDKDIYQLSESFISLLKLISFGAPGTFKFLGVEISQSNVRYQSVSSCFNATLIHQSITGLYETRIDLSKLGED

SEQ ID NO: 8 - protein, 1392 aa, Streptococcus mitis
MNNNNYSIGLDIGTNSVGWAVITDDYKVPSKKMKVLGNTDKHFIKKNLIGALLFDEGTTAEDRRLKRTARRRYTRRKNRLRYLQEIFSPEISKVDSSFFHRLDDSFLVPEDKRGSKYPIFATLAEEKEYHKNFPTIYHLRKQLADSKEKADLRLIYLALAHMIKYRGHFLYEESFDIKNNDIQKIFNEFISIYDNTFEGSSLSGQNAQVEAIFTDKISKSAKRERVLKLFPDEKSTGLFSEFLKLIVGNQAEFKKHFDLEEKAPLQFSKDTYDDDLENLLGQIGDGFAELFVAAKKLYDAILLSGILTVTDPSTKAPLSASMIERYENHQKDLAALKQFIQNNLQEKYDEVFSDQSKDGYAGYINGKTTQEAFYKYIKNLLSKFEGSDYFLDKIEREDFLKKQRTFDNGSIPHQIHLQEMNAIIRRQGEHYPFLQENKEKIKKILTFRIPYYVGPLARGNGDFAWLTRNSDQAIRPWNFEEIVDQASSAEDFINKMTNYDLYLPEEKVLPKHSLLYETFAVYNELTKVKFIAEGLRDYQFLDSGQKKQIVNQLFKEKRKVTEKDITQYLHNVDGYDGIELKGIEKQFNASLSTYHDLLKIIKDKAFMDDAENEATLENIIHTLTIFEDREMIKQRLAQYDSLFDEKVIKALIRRHYTGWGKLSAKLINGICDKKTGKTILDYLIDDGYSNRNFMQLINDDGLSFKDIIQKAQVVGRTNDVKQIVHELPGSPAIKKGILQSIKIVDELVKIMGHTPESIVIEMARENQTTARGKKNSQQRYKRIEDALKNLAPGLDSNILKEYPTDNIQLQNDRLFLYYLQNGKDMYTGEPLDINQLSSYDIDHIVPQAFIKDDSLDNRVLTSSKDNRGKSDNVPSLEVVQKRKAFWQQLLDSKLISERKFNNLTKAERGGLDERDKVGFIRRQLVETRQITKHVAQILDARFNTEVTEKDKKNRNVKIITLKSNLVSNFRKEFKLYKVREINDYHHAHDAYLNAVVAKAILKKYPKLEPEFVYGDYQKYDLKRYISRSKDPKDVEKATEKYFFYSNLLNFFKEEVHYADGTIVKRENIEYSKDTGEIAWNKEKDFATIKKVLSLPQVNIVKKTEIQTHGLDRGKPRGLFNSNPSPKPSEDSKENLVPIKQGLDPRKYGGYAGISNSYAVLVKAIIEKGAKKQQKTVLEFQGISILDKINFEKNKENYLLEKGYIKILSTITLPKYSLFEFPDGTRRRLASILSTNNKRGEIHKGNELVISEKYTTLLYHAKNINKTLEPEHLEYVEKHRNDFAKLLESVLDFNDKYVGALKNGERIRQAFIDWETVDIEKLCFSFIGPRNSKNAGLFELTSQGSASDFEFLGVKIPRYRDYTPSSLLNATLIHQSITGLYETRIDLSKLGED

SEQ ID NO: 9 - protein, 1334 aa, Listeria monocytogenes
MKNPYTIGLDIGTNSVGWAVLTDQYDLVKRKMKVAGNSDKKQIKKNFWGVRLFDEGETAADRRMNRTARRRIERRRNRISYLQEIFALEMANIDANFFCRLNDSFYVDSEKRNSRHPFFATIEEEVAYHKNYRTIYHLREELVNSSEKADLRLVYLALAHIIKYRGNFLIEGALDTKNTSVDGVYKQFIQTYNQVFISNIEEGTLAKMEENTTVADILAGKFTRKEKLERILQLYPGEKSTGMFAQFISLIVGSKGNFQKVFDLVEKTDIECAKDSYEEDLEALLAIIGDEYAELFVAAKNTYNAVVLSSIITVTDTETNAKLSASMIERFDAHEKDLSELKAFIKLHLPKQYEEIFSNVAIDGYAGYIDGKTKQVDFYKYLKTLLENIEGADYFIAKIEEENFLRKQRTFDNGAIPHQLHLEELEAILHQQAKYYPFLKEAYDKIKSLVTFRIPYFVGPLANGQSDFAWLTRKADGEIRPWNIEEKVDFGKSAVDFIEKMTNKDTYLPKENVLPKHSLYYQKYMVYNELTKVRYIDDQGKTNYFSGQEKQQIFNDYFKQKRKVSKKDLEQFLRNMSHIESPTIEGLEDSFNSSYATYHDLLKVGIKQEVLENPLNTEMLEDIVKILTVFEDKRMIKEQLQQFSDVLDGAVLKKLERRHYTGWGRLSAKLLVGIRDKQSHLTILDYLMNDDGLNRNLMQLINDSNLSFKSIIEKEQVSTTDKDLQSIVADLAGSPAIKKGILQSLKIVDELVSIMGYPPQTIVVEMARENQTTVKGKNNSRPRYKSLEKAIKEFGSQILKEHPTDNQELRNNRLYLYYLQNGKDMYTGQELDIHNLSNYDIDHIVPQSFITDNSIDNLVLTSSAGNREKGDDVPPLEIVRKRKVFWEKLFQGNLMSKRKFDYLTKAERGGLTEADKATFIHRQLVETRQITKNVANILHQRFNNETDNHGNNMEQVRIVMLKSALVSQFRKQFQLYKVREVNDYHHAHDAYLNGVVANTLLKVYPQLEPEFVYGEYHQFDWFKANKATAKKQFYTNIMLFFAQKERIIDENGEILWDKKYLETIKKVLDYRQMNIVKKTEIQKGEFSKATIKPKGNSSKLIPRKENWDPMKYGGLDSPNMAYAVIIEHAKGKKKVVFEKKIIRITIMERKAFEKDEKSFLEKQGYRQPKVLTKLPKYTLYECENGRRRMLASANEAQKGNQQVLKGQLITLLHHAKNCEASDGKSLDYIESNREMFGELLAHVSEFAKRYTLADANLSKINQLFEQNKDNDIKVIAQSFVNLMAFNAMGAPASFKFFEATIERKRYTNLKELLSATIIYQSITGLYEARKRLDG

SEQ ID NO: 10 - protein, 1342 aa, Enterococcus timonesis
MGKDYTIGLDIGTNSVGWAVLRDDLDLVKKKMKVFGNTDKKALKKNFWGVSLFDEGQTAADARMKRTMRRRLARRHQRIVFLQEEFFQKAMNEKDANFFHRLNESFLVEEDKEFNRHPIFGKLEEEKAYYKKYPTIYHLRKELADSTQQADLRLVYLAMAHIIKYRGHFLIEGKLSTENTSVSETFKVFLDKFNEASKIADNELKLDTTIDVEKVLTEKSSRSRKAENVLNFFPTEKKNDTFDQFLKMIVGNQGNFKKTFDLDEDAKLQFSKEDYDTELENLLGMAGDGYGDVFEAAKNAYNAVELSGILTVQDSLTKAKLSAGMIKRYDDHKEDLALLKKFFLNNLGYEEYVSYFKGDGKKDNNGYASYIDGHTKQDDFYSYTKKMLDKVEGADYFLAKIDQEDFLRKQRTFDNGVIPHQIHLEELKAIMEHQGEFYPFLKENFQKIVDLFNFRIPYYVGPLASKENHGRFAWLERNSDEPITPWNITEVVDMNKSAEKFIERMTNFDTYLPNEKVLPKHSMLYEKFTVYNELTKVSYTDEQEKTHNFSSIEKEKIFKELFCKNRKVTKDRLQKFLYNEYNLENVTINGIENEFNAKLATYHDFLKLNVSPEMLNDPENEDMFEEIVKMLTIFEDRKMLAKQLASFKSYFDEKTMKELVRRYYTGWGRLSAKLINGLYDQQTGKTVIDFLVMDDAPGKNTNRNFMQLINDNMLSFKEEIQKAQKEVGTKNDLNQIVQELAGSPALKKGILQSLKIVDEIVDIMGYAPTNIVIEMARENQTTGRGKINSQPRYKNLEKSLNEMQSKILKDYPTDNKAIQKDRLYLYYLQNGRDMYTGHDLDINNLSNYDIDHIIPQSFIVDNSIDNRVLVSSKENRGKSDDVLNIDIVKSRKGFWEQLLHSKLMSKKKFDNLTKAERGGITEDDKAGFIKRQLVETRQITKHVARILDERFNTEKDQTGKKIRTVRIVTLKSALTSQFRKNYQIYKVREINDYHHAHDAYLNGVVANTLLKIYPQLEPEFVYGEYHRYDSFKENRATAKKNMYSNIMQFTKKDVTLDKEGNGEILWDNKSVAMVKKVIDYRQMNIVKKTEIQRGGFSNETVLPKGPSDKLIPRKNNWDPAKYGGVGSPTEAYSIIISYEKGKSKKVVKEIVGITIMQRKAFEENELGFLKTRGYENPKVLAKLPKYTLFEFADGRRRLLASSKESQKGNQLVLSKDLNELVYHAKNSDKKSESLEFVTNNSTMFFDFLEYVDIFAQKYIIATKNSERIQIVAENNKDSEGKDLATSFFNLLQFTAMGAPADFKFFNETIPRKRYSSTSELLNATIIYQSVTGLYETRRNLGD

SEQ ID NO: 11 - protein, 1388 aa, Streptococcus thermophilus
MTKPYSIGLDIGTNSVGWAVTTDNYKVPSKKMKVLGNTSKKYIKKNLLGVLLFDSGITAEGRRLKRTARRRYTRRRNRILYLQEIFSTEMATLDDAFFQRLDDSFLVPDDKRDSKYPIFGNLVEEKAYHDEFPTIYHLRKYLADSTKKADLRLVYLALAHMIKYRGHFLIEGEFNSKNNDIQKNFQDFLDTYNAIFESDLSLENSKQLEEIVKDKISKLEKKDRILKLFPGEKNSGIFSEFLKLIVGNQADFRKCFNLDEKASLHFSKESYDEDLETLLGYIGDDYSDVFLKAKKLYDAILLSGFLTVTDNETEAPLSSAMIKRYNEHKEDLALLKEYIRNISLKTYNEVFKDDTKNGYAGYIDGKTNQEDFYVYLKKLLAKFEGADYFLEKIDREDFLRKQRTFDNGSIPYQIHLQEMRAILDKQAKFYPFLAKNKERIEKILTFRIPYYVGPLARGNSDFAWSIRKRNEKITPWNFEDVIDKESSAEAFINRMTSFDLYLPEEKVLPKHSLLYETFNVYNELTKVRFIAESMRDYQFLDSKQKKDIVRLYFKDKRKVTDKDIIEYLHAIYGYDGIELKGIEKQFNSSLSTYHDLLNIINDKEFLDDSSNEAIIEEIIHTLTIFEDREMIKQRLSKFENIFDKSVLKKLSRRHYTGWGKLSAKLINGIRDEKSGNTILDYLIDDGISNRNFMQLIHDDALSFKKKIQKAQIIGDEDKGNIKEVVKSLPGSPAIKKGILQSIKIVDELVKVMGGRKPESIVVEMARENQYTNQGKSNSQQRLKRLEKSLKELGSKILKENIPAKLSKIDNNALQNDRLYLYYLQNGKDMYTGDDLDIDRLSNYDIDHIIPQAFLKDNSIDNKVLVSSASNRGKSDDVPSLEVVKKRKTFWYQLLKSKLISQRKFDNLTKAERGGLSPEDKAGFIQRQLVETRQITKHVARLLDEKFNNKKDENNRAVRTVKIITLKSTLVSQFRKDFELYKVREINDFHHAHDAYLNAVVASALLKKYPKLEPEFVYGDYPKYNSFRERKSATEKVYFYSNIMNIFKKSISLADGRVIERPLIEVNEETGESVWNKESDLATVRRVLSYPQVNVVKKVEEQNHGLDRGKPKGLFNANLSSKPKPNSNENLVGAKEYLDPKKYGGYAGISNSFAVLVKGTIEKGAKKKITNVLEFQGISILDRINYRKDKLNFLLEKGYKDIELIIELPKYSLFELSDGSRRMLASILSTNNKRGEIHKGNQIFLSQKFVKLLYHAKRISNTINENHRKYVENHKKEFEELFYYILEFNENYVGAKKNGKLLNSAFQSWQNHSIDELCSSFIGPTGSERKGLFELTSRGSAADFEFLGVKIPRYRDYTPSSLLKDATLIHQSVTGLYETRIDLAKLGEG

SEQ ID NO: 12 - protein, 1366 aa, Streptococcus parasanguinis
MKKPYSIGLDIGTNSVGWAVITDDYKVPAKKMKVLGNTNKESIKKNLIGALLFDAGNTAADRRLKRTARRRYTRRRNRILYLQEIFAAEMNKVDESFFHRLDDSFLVPEDKRGSKYPIFGTLEEEKEYHKQFPTIYYLRKILADSKEKVDLRLIYLALAHIIKYRGHFLYEDSFDIKNNDIQKIFNEFTILYDNTFEESSLSKGNAQVEEIFTDKISKSAKRDRVLKLFPDEKSTGLFSEFLKLIVGNQADFKKHFDLEEKAPLQFSKDTYEEDLESLLGQIGDVYADLFVVAKKLYDAILLAGILSVKDPGTKAPLSASMIERYDNHQNDLSALKQFVRRNLPEKYAEVFSDDSKDGYAGYIDGKTTQEGFYKYIKNLISKIEGAEYFLEKIEREDFLRKQRTFDNGSIPHQIHLQEMNAILRHQGEYYPFLKENKDKIEQILTFRIPYYVGPLARGNSDFAWLSRNSDEAIRPWNFEEMVDKSSSAEDFIHRMTNYDLYLPEEKVLPKHSLLYETFTVYNELTKVKYIAEGMKDYQFLDSGQKKQIVNQLFKEKRKVTEKDIIHYLHNVDGYDGIELKGIEKHFNSSLSTYHDLLKIIKDKEFMDDPKNEEIFENIVHTLTIFEDRVMIKQRLNQYDSIFDEKVIKALTRRHYTGWGKLSAKLINGIRDKKTSKTILDYLIDDGYSNRNFMQLINDDGLSFKETIQKAQVVGETNDVKQVVQELPGSPAIKKGILQSIKIVDELVKVMGHAPESVVIEMARENQTTNKGKSKSQQRLKTLSDAISELGSNILKEHPTDNIQLQNDRLFLYYLQNGKDMYTGEALDINQLSNYDIDHIIPQAFIKDDSLDNRVLTSSKDNRGKSDNVPSLEIVEKMKGFWQQLLDSKLISERKFNNLTKAERGGLDERDKVGFIKRQLVETRQITKHVAQILDDRFNAEVNEKNQKLRSVKIITLKSNLVSNFRKEFGLYKVREINDYHHAHDAYLNAVVAKAILKKYPKLEPEFVYGDYQKYDLKRYISRTKDPKEIEKATEKYFFYSNLLNFFKDKVYYADGTIIQRGNVEYSKDTGEIAWNKKRDFAIVRKVLSYPQVNIVKKTEEQTGGFSKESILPKGNSDKLIPRKTKNVQLDTTKYGGFDSPVIAYSILLVADVEKGKSKKLKTVKSLIGITIMEKVKFEANPVAFLEGKGYQNVVEENIIRLPKYSLFELENGRRRMLASAKELQKGNEMVLPSYLIALLYHAKRIQKKDEPEHLEYIKQHHSEFNDLLNFVSEFSQKYVLAESNLEKIKNLYIDNEQTNMEEIANSFINLLTFTAFGAPAVFKFFGKDIERKRYSTVTEILKATLIHQSLTGLYETRIDLSKLGEE

SEQ ID NO: 13 - protein, 1368 aa, synthetic construct
  REGION 1..1368: note = Base sequence SEQ ID NO: 1, residues 695, 848, and 926 substituted with Alanine, residue 923 substituted with Methionine, and residue 924 substituted with Valine
MDKKYSIGLDIGTNSVGWAVITDEYKVPSKKFKVLGNTDRHSIKKNLIGALLFDSGETAEATRLKRTARRRYTRRKNRICYLQEIFSNEMAKVDDSFFHRLEESFLVEEDKKHERHPIFGNIVDEVAYHEKYPTIYHLRKKLVDSTDKADLRLIYLALAHMIKFRGHFLIEGDLNPDNSDVDKLFIQLVQTYNQLFEENPINASGVDAKAILSARLSKSRRLENLIAQLPGEKKNGLFGNLIALSLGLTPNFKSNFDLAEDAKLQLSKDTYDDDLDNLLAQIGDQYADLFLAAKNLSDAILLSDILRVNTEITKAPLSASMIKRYDEHHQDLTLLKALVRQQLPEKYKEIFFDQSKNGYAGYIDGGASQEEFYKFIKPILEKMDGTEELLVKLNREDLLRKQRTFDNGSIPHQIHLGELHAILRRQEDFYPFLKDNREKIEKILTFRIPYYVGPLARGNSRFAWMTRKSEETITPWNFEEVVDKGASAQSFIERMTNFDKNLPNEKVLPKHSLLYEYFTVYNELTKVKYVTEGMRKPAFLSGEQKKAIVDLLFKTNRKVTVKQLKEDYFKKIECFDSVEISGVEDRFNASLGTYHDLLKIIKDKDFLDNEENEDILEDIVLTLTLFEDREMIEERLKTYAHLFDDKVMKQLKRRRYTGWGRLSRKLINGIRDKQSGKTILDFLKSDGFANRNFMALIHDDSLTFKEDIQKAQVSGQGDSLHEHIANLAGSPAIKKGILQTVKVVDELVKVMGRHKPENIVIEMARENQTTQKGQKNSRERMKRIEEGIKELGSQILKEHPVENTQLQNEKLYLYYLQNGRDMYVDQELDINRLSDYDVDHIVPQSFLADDSIDNKVLTRSDKNRGKSDNVPSEEVVKKMKNYWRQLLNAKLITQRKFDNLTKAERGGLSELDKAGFIKRQLVMVRAITKHVAQILDSRMNTKYDENDKLIREVKVITLKSKLVSDFRKDFQFYKVREINNYHHAHDAYLNAVVGTALIKKYPKLESEFVYGDYKVYDVRKMIAKSEQEIGKATAKYFFYSNIMNFFKTEITLANGEIRKRPLIETNGETGEIVWDKGRDFATVRKVLSMPQVNIVKKTEVQTGGFSKESILPKRNSDKLIARKKDWDPKKYGGFDSPTVAYSVLVVAKVEKGKSKKLKSVKELLGITIMERSSFEKNPIDFLEAKGYKEVKKDLIIKLPKYSLFELENGRKRMLASAGELQKGNELALPSKYVNFLYLASHYEKLKGSPEDNEQKQLFVEQHKHYLDEIIEQISEFSKRVILADANLDKVLSAYNKHRDKPIREQAENIIHLFTLTNLGAPAAFKYFDTTIDRKRYTSTKEVLDATLIHQSITGLYETRIDLSQLGGD

SEQ ID NO: 14 - DNA, 47 bp, synthetic construct
  misc_feature 1..47: note = forward primer
  source 1..47: mol_type = other DNA
aatgatacggcgaccaccgagatctacacggaaccgcaacggtattc

SEQ ID NO: 15 - DNA, 52 bp, synthetic construct
  misc_feature 1..52: note = reverse primer
  misc_feature 25..32: note = NNNNNNNN denotes a specific indexing barcode assigned for each experimental sample
  source 1..52: mol_type = other DNA
caagcagaagacggcatacgagatnnnnnnnnggttgcgtcagcaaacacag

SEQ ID NO: 16 - DNA, 20 bp, synthetic construct
  misc_feature 1..20: note = quantitative PCR forward primer
  source 1..20: mol_type = other DNA
aatgatacggcgaccaccga

SEQ ID NO: 17 - DNA, 21 bp, synthetic construct
  misc_feature 1..21: note = quantitative PCR reverse primer
  source 1..21: mol_type = other DNA
caagcagaagacggcatacga

SEQ ID NO: 18 - DNA, 34 bp, synthetic construct
  misc_feature 1..34: note = Illumina HiSeq primer
  source 1..34: mol_type = other DNA
ccaccgagatctacacggaaccgcaacggtattc

SEQ ID NO: 19 - DNA, 35 bp, synthetic construct
  misc_feature 1..35: note = indexing barcode primer
  source 1..35: mol_type = other DNA
gtggcgtggtgtgcactgtgtttgctgacgcaacc

SEQ ID NO: 20 - DNA, 34 bp, synthetic construct
  misc_feature 1..34: note = dsODN oligonucleotide
  misc_feature 1: note = 5' phosphorylation
  misc_feature 1..2: note = phosphorothioate linkage
  misc_feature 2..3: note = phosphorothioate linkage
  misc_feature 32..33: note = phosphorothioate linkage
  misc_feature 33..34: note = phosphorothioate linkage
  source 1..34: mol_type = other DNA
gtttaattgagttgtcatatgttaataacggtat

SEQ ID NO: 21 - DNA, 34 bp, synthetic construct
  misc_feature 1..34: note = dsODN oligonucleotide
  misc_feature 1: note = 5' phosphorylation
  misc_feature 1..2: note = phosphorothioate linkage
  misc_feature 2..3: note = phosphorothioate linkage
  misc_feature 32..33: note = phosphorothioate linkage
  misc_feature 33..34: note = phosphorothioate linkage
  source 1..34: mol_type = other DNA
ataccgttattaacatatgacaactcaattaaac

SEQ ID NO: 22 - DNA, 20 bp, synthetic construct
  misc_feature 1..20: note = BRD4sg3 gN20 sgRNA protospacer
  source 1..20: mol_type = other DNA
gggaacaataaagaagcgct

SEQ ID NO: 23 - DNA, 20 bp, synthetic construct
  misc_feature 1..20: note = KDM4Csg1 gN20 sgRNA protospacer
  source 1..20: mol_type = other DNA
cctttgcaagacccgcacga

SEQ ID NO: 24 - DNA, 20 bp, synthetic construct
  misc_feature 1..20: note = PRMT2sg3 gN20 sgRNA protospacer
  source 1..20: mol_type = other DNA
ctgtcccagaagtgaatcgc

SEQ ID NO: 25 - DNA, 20 bp, synthetic construct
  misc_feature 1..20: note = HDAC2sg1 gN20 sgRNA protospacer
  source 1..20: mol_type = other DNA
tccgtaatgttgctcgatgt

SEQ ID NO: 26 - DNA, 20 bp, synthetic construct
  misc_feature 1..20: note = PRMT6sg1 GN20 sgRNA protospacer
  source 1..20: mol_type = other DNA
attgtccggcgaggacgtgc

SEQ ID NO: 27 - DNA, 20 bp, synthetic construct
  misc_feature 1..20: note = NF1sg1 gN20 sgRNA protospacer
  source 1..20: mol_type = other DNA
gttgtgctcagtactgactt

SEQ ID NO: 28 - DNA, 20 bp, synthetic construct
  misc_feature 1..20: note = NF2sg1 GN20 sgRNA protospacer
  source 1..20: mol_type = other DNA
aaacatctcgtacagtgaca

SEQ ID NO: 29 - DNA, 20 bp, synthetic construct
  misc_feature 1..20: note = VEGFAsg-site3 GN20 sgRNA protospacer
  source 1..20: mol_type = other DNA
ggtgagtgagtgtgtgcgtg

SEQ ID NO: 30 - DNA, 20 bp, synthetic construct
  misc_feature 1..20: note = DNMT1sg-site 4 GN20 protospacer
  source 1..20: mol_type = other DNA
ggagtgagggaaacggcccc

SEQ ID NO: 31 - DNA, 20 bp, synthetic construct
  misc_feature 1..20: note = FANCFsg-site 6 gN20 sgRNA protospacer
  source 1..20: mol_type = other DNA
gcttgagaccgccagaagct

SEQ ID NO: 32 - DNA, 20 bp, synthetic construct
  misc_feature 1..20: note = EMX1sg-site 3 gN20 sgRNA protospacer
  source 1..20: mol_type = other DNA
gagtccgagcagaagaagaa

SEQ ID NO: 33 - DNA, 20 bp, synthetic construct
  misc_feature 1..20: note = CXCR4sg GN20 sgRNA protospacer
  source 1..20: mol_type = other DNA
gaagcgtgatgacaaagagg

SEQ ID NO: 34 - DNA, 20 bp, synthetic construct
  misc_feature 1..20: note = PD1sg gN20 sgRNA protospacer
  source 1..20: mol_type = other DNA
ggccaggatggttcttaggt

SEQ ID NO: 35 - DNA, 20 bp, synthetic construct
  misc_feature 1..20: note = EMX1sg site 2 gN20 sgRNA protospacer
  source 1..20: mol_type = other DNA
gtcacctccaatgactaggg

SEQ ID NO: 36 - DNA, 20 bp, synthetic construct
  misc_feature 1..20: note = FANCFsg-site 3 gN20 sgRNA protospacer
  source 1..20: mol_type = other DNA
ggcggctgcacaaccagtgg

SEQ ID NO: 37 - DNA, 20 bp, synthetic construct
  misc_feature 1..20: note = ZSCAN2sg gN20 sgRNA protospacer
  source 1..20: mol_type = other DNA
gtgcggcaagagcttcagcc

SEQ ID NO: 38 - DNA, 20 bp, synthetic construct
  misc_feature 1..20: note = FANCFsg-Site 1 gN20 sgRNA protospacer
  source 1..20: mol_type = other DNA
ggaatcccttctgcagcacc

SEQ ID NO: 39 - DNA, 20 bp, synthetic construct
  misc_feature 1..20: note = RUNXsg-Site 1 gN20 sgRNA protospacer
  source 1..20: mol_type = other DNA
gcattttcaggaggaagcga

SEQ ID NO: 40 - DNA, 20 bp, synthetic construct
  misc_feature 1..20: note = EMX1sg1 GN20 sgRNA protospacer
  source 1..20: mol_type = other DNA
gcctccccaaagcctggcca

SEQ ID NO: 41 - DNA, 20 bp, synthetic construct
  misc_feature 1..20: note = DMDsg gN20 sgRNA protospacer
  source 1..20: mol_type = other DNA
ctttctacctactgagtctg

SEQ ID NO: 42 - DNA, 20 bp, synthetic construct
  misc_feature 1..20: note = AAVSsg gN20 sgRNA protospacer
  source 1..20: mol_type = other DNA
ctccctcccaggatcctctc

SEQ ID NO: 43 - DNA, 20 bp, synthetic construct
  misc_feature 1..20: note = HPRTsg gN20 sgRNA protospacer
  source 1..20: mol_type = other DNA
tcgagatgtgatgaaggaga

SEQ ID NO: 44 - DNA, 20 bp, synthetic construct
  misc_feature 1..20: note = HPRT38087sg gN20 sgRNA protospacer
  source 1..20: mol_type = other DNA
aattatggggattactagga

SEQ ID NO: 45 - DNA, 20 bp, synthetic construct
  misc_feature 1..20: note = FANCFsg-site 2 GN19 sgRNA protospacer
  source 1..20: mol_type = other DNA
gctgcagaagggattccatg

SEQ ID NO: 46 - DNA, 20 bp, synthetic construct
  misc_feature 1..20: note = FANCFsg-site 6 GN19 sgRNA protospacer
  source 1..20: mol_type = other DNA
gcttgagaccgccagaagct

SEQ ID NO: 47 - DNA, 20 bp, synthetic construct
  misc_feature 1..20: note = EMX1sg-site 3 GN19 sgRNA protospacer
  source 1..20: mol_type = other DNA
gagtccgagcagaagaagaa

SEQ ID NO: 48 - DNA, 20 bp, synthetic construct
  misc_feature 1..20: note = DNMT1sg-site 4 GN19 sgRNA protospacer
  source 1..20: mol_type = other DNA
ggagtgagggaaacggcccc

SEQ ID NO: 49 - DNA, 20 bp, synthetic construct
  misc_feature 1..20: note = NF1sg1 GN19 sgRNA protospacer
  source 1..20: mol_type = other DNA
gttgtgctcagtactgactt

SEQ ID NO: 50 - DNA, 20 bp, synthetic construct
  misc_feature 1..20: note = CXCR4sg GN19 sgRNA protospacer
  source 1..20: mol_type = other DNA
gaagcgtgatgacaaagagg

SEQ ID NO: 51 - DNA, 20 bp, synthetic construct
  misc_feature 1..20: note = PD1sg GN19 sgRNA protospacer
  source 1..20: mol_type = other DNA
ggccaggatggttcttaggt

SEQ ID NO: 52 - DNA, 20 bp, synthetic construct
  misc_feature 1..20: note = EMX1sg-site 2 GN19 sgRNA protospacer
  source 1..20: mol_type = other DNA
gtcacctccaatgactaggg

SEQ ID NO: 53 - DNA, 20 bp, synthetic construct
  misc_feature 1..20: note = ZSCAN2sg GN19 sgRNA protospacer
  source 1..20: mol_type = other DNA
gtgcggcaagagcttcagcc

SEQ ID NO: 54 - DNA, 20 bp, synthetic construct
  misc_feature 1..20: note = FANCFsg Site 1 GN19 sgRNA protospacer
  source 1..20: mol_type = other DNA
ggaatcccttctgcagcacc

SEQ ID NO: 55 - DNA, 20 bp, synthetic construct
  misc_feature 1..20: note = RUNXsg Site 1 GN19 sgRNA protospacer
  source 1..20: mol_type = other DNA
gcattttcaggaggaagcga

SEQ ID NO: 56 - DNA, 20 bp, synthetic construct
  misc_feature 1..20: note = EMX1sg1 GN19 sgRNA protospacer
  source 1..20: mol_type = other DNA
gcctccccaaagcctggcca

SEQ ID NO: 57 - DNA, 20 bp, synthetic construct
  misc_feature 1..20: note = BRD4sg3 GN19 sgRNA protospacer
  source 1..20: mol_type = other DNA
gggaacaataaagaagcgct

SEQ ID NO: 58 - DNA, 19 bp, synthetic construct
  misc_feature 1..19: note = PRMT2sg3 gN19 sgRNA protospacer
  source 1..19: mol_type = other DNA
tgtcccagaagtgaatcgc

SEQ ID NO: 59 - DNA, 19 bp, synthetic construct
  misc_feature 1..19: note = KDM4Csg1 gN19 sgRNA protospacer
  source 1..19: mol_type = other DNA
ctttgcaagacccgcacga

SEQ ID NO: 60 - DNA, 19 bp, synthetic construct
  misc_feature 1..19: note = HDAC2sg1 gN19 sgRNA protospacer
  source 1..19: mol_type = other DNA
ccgtaatgttgctcgatgt

SEQ ID NO: 61 - DNA, 19 bp, synthetic construct
  misc_feature 1..19: note = HPRTsg gN19 sgRNA protospacer
  source 1..19: mol_type = other DNA
cgagatgtgatgaaggaga

SEQ ID NO: 62 - DNA, 19 bp, synthetic construct
  misc_feature 1..19: note = HPRT38087sg gN19 sgRNA protospacer
  source 1..19: mol_type = other DNA
attatggggattactagga

SEQ ID NO: 63 - DNA, 19 bp, synthetic construct
  misc_feature 1..19: note = DNMT1sg-site 4-19nt
  source 1..19: mol_type = other DNA
gagtgagggaaacggcccc

SEQ ID NO: 64 - DNA, 17 bp, synthetic construct
  misc_feature 1..17: note = DNMT1sg-site 4-17nt sgRNA protospacer
  source 1..17: mol_type = other DNA
gtgagggaaacggcccc

SEQ ID NO: 65 - DNA, 18 bp, synthetic construct
  misc_feature 1..18: note = PRMT2sg3-18nt sgRNA sequence
  source 1..18: mol_type = other DNA
gtcccagaagtgaatcgc

SEQ ID NO: 66 - DNA, 18 bp, synthetic construct
  misc_feature 1..18: note = EMX1-site 3-18nt sgRNA protospacer
  source 1..18: mol_type = other DNA
gtccgagcagaagaagaa

SEQ ID NO: 67 - DNA, 19 bp, synthetic construct
  misc_feature 1..19: note = BRD4sg3-19nt sgRNA protospacer
  source 1..19: mol_type = other DNA
ggaacaataaagaagcgct

SEQ ID NO: 68 - DNA, 18 bp, synthetic construct
  misc_feature 1..18: note = BRD4sg3-18nt sgRNA protospacer
  source 1..18: mol_type = other DNA
gaacaataaagaagcgct

SEQ ID NO: 69 - DNA, 20 bp, synthetic construct
  misc_feature 1..20: note = RFPsg5 sgRNA protospacer
  source 1..20: mol_type = other DNA
cacccagaccatgaagatca

SEQ ID NO: 70 - DNA, 20 bp, synthetic construct
  misc_feature 1..20: note = RFPsg6 sgRNA protospacer
  source 1..20: mol_type = other DNA
ccacttcaagtgcacatccg

SEQ ID NO: 71 - DNA, 20 bp, synthetic construct
  misc_feature 1..20: note = RFPsg8 sgRNA protospacer
  source 1..20: mol_type = other DNA
ctggctaccagcttcatgta

SEQ ID NO: 72 - DNA, 20 bp, synthetic construct
  misc_feature 1..20: note = GFPsg1 sgRNA protospacer
  source 1..20: mol_type = other DNA
gggcgaggagctgttcaccg

SEQ ID NO: 73 - DNA, 20 bp, synthetic construct
  misc_feature 1..20: note = GFPsg1-2MM1 sgRNA protospacer
  source 1..20: mol_type = other DNA
gggtgaggagctgtttaccg

SEQ ID NO: 74 - DNA, 20 bp, synthetic construct
  misc_feature 1..20: note = GFPsg1-2MM3 sgRNA protospacer
  source 1..20: mol_type = other DNA
gggtgacgagctgttcaccg

SEQ ID NO: 75 - DNA, 20 bp, synthetic construct
  misc_feature 1..20: note = GFPsg1-2MM6 sgRNA protospacer
  source 1..20: mol_type = other DNA
gggcgaggagcagatcaccg

SEQ ID NO: 76 - DNA, 20 bp, synthetic construct
  misc_feature 1..20: note = GFPsg1-2MM8 sgRNA protospacer
  source 1..20: mol_type = other DNA
gtgcgaggagctgttcgccg

SEQ ID NO: 77 - DNA, 20 bp, synthetic construct
  misc_feature 1..20: note = GFPsg1-2MM9 sgRNA protospacer
  source 1..20: mol_type = other DNA
gagcgagtagctgttcaccg

SEQ ID NO: 78 - DNA, 20 bp, synthetic construct
  misc_feature 1..20: note = GFPsg1-2MM10 sgRNA protospacer
  source 1..20: mol_type = other DNA
gggagaggagctgtgcaccg

SEQ ID NO: 79 - DNA, 20 bp, synthetic construct
  misc_feature 1..20: note = GFPsg1-2MM13 sgRNA protospacer
  source 1..20: mol_type = other DNA
gggccaggaggtgttcaccg

SEQ ID NO: 80 - DNA, 20 bp, synthetic construct
  misc_feature 1..20: note = GFPsg1-2MM14 sgRNA protospacer
  source 1..20: mol_type = other DNA
gggcgaggtgctattcaccg

SEQ ID NO: 81 - DNA, 20 bp, synthetic construct
  misc_feature 1..20: note = GFPsg1-3MM5 sgRNA protospacer
  source 1..20: mol_type = other DNA
tggggaggagctgttcaccc

SEQ ID NO: 82 - DNA, 20 bp, synthetic construct
  misc_feature 1..20: note = GFPsg1-3MM6 sgRNA protospacer
  source 1..20: mol_type = other DNA
ggacgcggatctgttcaccg

SEQ ID NO: 83 - DNA, 20 bp, synthetic construct
  misc_feature 1..20: note = GFPsg1-3MM8 sgRNA protospacer
  source 1..20: mol_type = other DNA
gggcgggcagcggttcaccg

SEQ ID NO: 84 - DNA, 20 bp, synthetic construct
  misc_feature 1..20: note = GFPsg1-4MM1
  source 1..20: mol_type = other DNA
gggccatgagctggttaccg

SEQ ID NO: 85 - DNA, 20 bp, synthetic construct
  misc_feature 1..20: note = GFPsg1-4MM5 sgRNA protospacer
  source 1..20: mol_type = other DNA
gggcgcgaagcatttcaccg

SEQ ID NO: 86 - DNA, 20 bp, synthetic construct
  misc_feature 1..20: note = GFPsg1-4MM6 sgRNA protospacer
  source 1..20: mol_type = other DNA
gggacagcagcagttcaccg

SEQ ID NO: 87 - DNA, 20 bp, synthetic construct
  misc_feature 1..20: note = GFPsg1-4MM8 sgRNA protospacer
  source 1..20: mol_type = other DNA
ggaggacgagctgctcaccg

SEQ ID NO: 88 - DNA, 20 bp, synthetic construct
  misc_feature 1..20: note = GFPsg1-M1 sgRNA protospacer
  source 1..20: mol_type = other DNA
gggcgaggagctgttcacca

SEQ ID NO: 89 - DNA, 20 bp, synthetic construct
  misc_feature 1..20: note = GFPsg1-M2 sgRNA protospacer
  source 1..20: mol_type = other DNA
gggcgaggagctgttcactg

SEQ ID NO: 90 - DNA, 20 bp, synthetic construct
  misc_feature 1..20: note = GFPsg1-M3 sgRNA protospacer
  source 1..20: mol_type = other DNA
gggcgaggagctgttcatcg

SEQ ID NO: 91 - DNA, 20 bp, synthetic construct
  misc_feature 1..20: note = GFPsg1-M4 sgRNA protospacer
  source 1..20: mol_type = other DNA
gggcgaggagctgttcgccg

SEQ ID NO: 92 - DNA, 20 bp, synthetic construct
  misc_feature 1..20: note = GFPsg1-M5 sgRNA protospacer
  source 1..20: mol_type = other DNA
gggcgaggagctgtttaccg

SEQ ID NO: 93 - DNA, 20 bp, synthetic construct
  misc_feature 1..20: note = GFPsg1-M6 sgRNA protospacer
  source 1..20: mol_type = other DNA
gggcgaggagctgtccaccg

SEQ ID NO: 94 - DNA, 20 bp, synthetic construct
  misc_feature 1..20: note = GFPsg1-M7 sgRNA protospacer
  source 1..20: mol_type = other DNA
gggcgaggagctgctcaccg

SEQ ID NO: 95 - DNA, 20 bp, synthetic construct
  misc_feature 1..20: note = GFPsg1-M8 sgRNA protospacer
  source 1..20: mol_type = other DNA
gggcgaggagctattcaccg

SEQ ID NO: 96 - DNA, 20 bp, synthetic construct
  misc_feature 1..20: note = GFPsg1-M9 sgRNA protospacer
  source 1..20: mol_type = other DNA
gggcgaggagccgttcaccg

SEQ ID NO: 97 - DNA, 20 bp, synthetic construct
  misc_feature 1..20: note = GFPsg1-M10 sgRNA protospacer
  source 1..20: mol_type = other DNA
gggcgaggagttgttcaccg

SEQ ID NO: 98 - DNA, 20 bp, synthetic construct
  misc_feature 1..20: note = GFPsg1-M11 sgRNA protospacer
  source 1..20: mol_type = other DNA
gggcgaggaactgttcaccg

SEQ ID NO: 99 - DNA, 20 bp, synthetic construct
  misc_feature 1..20: note = GFPsg1-M12 sgRNA protospacer
  source 1..20: mol_type = other DNA
gggcgaggggctgttcaccg

SEQ ID NO: 100 - DNA, 20 bp, synthetic construct
  misc_feature 1..20: note = GFPsg1-M13 sgRNA protospacer
  source 1..20: mol_type = other DNA
gggcgagaagctgttcaccg

SEQ ID NO: 101 - DNA, 20 bp, synthetic construct
  misc_feature 1..20: note = GFPsg1-M14 sgRNA protospacer
  source 1..20: mol_type = other DNA
gggcgaagagctgttcaccg

SEQ ID NO: 102 - DNA, 20 bp, synthetic construct
  misc_feature 1..20: note = GFPsg1-M15 sgRNA protospacer
  source 1..20: mol_type = other DNA
gggcggggagctgttcaccg

SEQ ID NO: 103 - DNA, 20 bp, synthetic construct
  misc_feature 1..20: note = GFPsg1-M16 sgRNA protospacer
  source 1..20: mol_type = other DNA
gggcaaggagctgttcaccg

SEQ ID NO: 104 - DNA, 20 bp, synthetic construct
  misc_feature 1..20: note = GFPsg1-M17 sgRNA protospacer
  source 1..20: mol_type = other DNA
gggtgaggagctgttcaccg

SEQ ID NO: 105 - DNA, 20 bp, synthetic construct
  misc_feature 1..20: note = GFPsg1-M18 sgRNA protospacer
  source 1..20: mol_type = other DNA
ggacgaggagctgttcaccg

SEQ ID NO: 106 - DNA, 20 bp, synthetic construct
  misc_feature 1..20: note = GFPsg1-M19 sgRNA protospacer
  source 1..20: mol_type = other DNA
gagcgaggagctgttcaccg

SEQ ID NO: 107 - DNA, 20 bp, synthetic construct
  misc_feature 1..20: note = GFPsg1-M20 sgRNA protospacer
  source 1..20: mol_type = other DNA
aggcgaggagctgttcaccg

SEQ ID NO: 108 - DNA, 20 bp, synthetic construct
  misc_feature 1..20: note = GFP-site20 sgRNA protospacer
  source 1..20: mol_type = other DNA
gaagttcgagggcgacaccc

SEQ ID NO: 109 - DNA, 20 bp, synthetic construct
  misc_feature 1..20: note = GFP 5'-G site20 sgRNA protospacer
  source 1..20: mol_type = other DNA
gaagttcgagggcgacaccc

SEQ ID NO: 110 - DNA, 20 bp, synthetic construct
  misc_feature 1..20: note = GFP-site25 sgRNA protospacer
  source 1..20: mol_type = other DNA
cctcgaacttcacctcggcg

SEQ ID NO: 111 - DNA, 20 bp, synthetic construct
  misc_feature 1..20: note = GFP 5'-G site25 sgRNA protospacer
  source 1..20: mol_type = other DNA
cctcgaacttcacctcggcg

SEQ ID NO: 112 - DNA, 20 bp, synthetic construct
  misc_feature 1..20: note = GFP 5'-C sgRNA protospacer
  source 1..20: mol_type = other DNA
ctcgtgaccaccctgaccta

SEQ ID NO: 113 - DNA, 20 bp, synthetic construct
  misc_feature 1..20: note = GFP 5'-GC sgRNA protospacer
  source 1..20: mol_type = other DNA
ctcgtgaccaccctgaccta

SEQ ID NO: 114 - DNA, 20 bp, synthetic construct
  misc_feature 1..20: note = GFP 5'-A sgRNA protospacer
  source 1..20: mol_type = other DNA
accatcttcttcaaggacga

SEQ ID NO: 115 - DNA, 20 bp, synthetic construct
  misc_feature 1..20: note = GFP 5'-GA sgRNA protospacer
  source 1..20: mol_type = other DNA
accatcttcttcaaggacga

SEQ ID NO: 116 - DNA, 19 bp, synthetic construct
  misc_feature 1..19: note = GFPon-19nt sgRNA protospacer
  source 1..19: mol_type = other DNA
ggcacgggcagcttgccgg

SEQ ID NO: 117 - DNA, 18 bp, synthetic construct
  misc_feature 1..18: note = GFPB-18nt sgRNA protospacer
  source 1..18: mol_type = other DNA
ggcaagctgcccgtgccc

SEQ ID NO: 118 - DNA, 17 bp, synthetic construct
  misc_feature 1..17: note = GFPW-17nt sgRNA protospacer
  source 1..17: mol_type = other DNA
gtgaccaccctgaccta

SEQ ID NO: 119 - DNA, 20 bp, synthetic construct
  misc_feature 1..20: note = RFPsg5-ON target sequence on RFP
  source 1..20: mol_type = other DNA
cacccagaccatgaagatca

SEQ ID NO: 120 - DNA, 20 bp, synthetic construct
  misc_feature 1..20: note = RFPsg5-OFF5 target sequence on RFP
  source 1..20: mol_type = other DNA
gacccaaaccatgaagatca

SEQ ID NO: 121 - DNA, 20 bp, synthetic construct
  misc_feature 1..20: note = RFPsg5-OFF5-2 target sequence on RFP
  source 1..20: mol_type = other DNA
cacccaaaccatgaagatca

SEQ ID NO: 122 - DNA, 20 bp, synthetic construct
  misc_feature 1..20: note = RFPsg6-ON target sequence on RFP
  source 1..20: mol_type = other DNA
ccacttcaagtgcacatccg

SEQ ID NO: 123 - DNA, 20 bp, synthetic construct
  misc_feature 1..20: note = RFPsg8-ON target sequence on RFP
  source 1..20: mol_type = other DNA
ctggctaccagcttcatgta

SEQ ID NO: 124 - DNA, 20 bp, synthetic construct
  misc_feature 1..20: note = RFPsg8-OFF5 target sequence on RFP
  source 1..20: mol_type = other DNA
gtgcctccctgcttcatgta

SEQ ID NO: 125 - DNA, 22 bp, synthetic construct
  misc_feature 1..22: note = BRD4 Forward Primer
  source 1..22: mol_type = other DNA
cacttgctgatgccagtaggag

SEQ ID NO: 126 - DNA, 22 bp, synthetic construct
  misc_feature 1..22: note = BRD4 reverse primer
  source 1..22: mol_type = other DNA
aagcacatgcttcaggctaaca

SEQ ID NO: 127 - DNA, 22 bp, synthetic construct
  misc_feature 1..22: note = DNMT1 site 4 forward primer
  source 1..22: mol_type = other DNA
ccacttgacaggcgagtaacag

SEQ ID NO: 128 - DNA, 18 bp, synthetic construct
  misc_feature 1..18: note = DNMT1 site 4 reverse primer
  source 1..18: mol_type = other DNA
ccaaggatcttgtgctgg

SEQ ID NO: 129 - DNA, 20 bp, synthetic construct
  misc_feature 1..20: note = DNMT1 site 4 OFF1 forward primer
  source 1..20: mol_type = other DNA
ccaacaagccctaaccagga

SEQ ID NO: 130 - DNA, 20 bp, synthetic construct
  misc_feature 1..20: note = DNMT1 site 4 OFF1 reverse primer
  source 1..20: mol_type = other DNA
agaacgagaatgctcggcag

SEQ ID NO: 131 - DNA, 22 bp, synthetic construct
  misc_feature 1..22: note = HDAC2 forward primer
  source 1..22: mol_type = other DNA
gacttttccatcagggacacct

SEQ ID NO: 132 - DNA, 24 bp, synthetic construct
  misc_feature 1..24: note = HDAC2 reverse primer
  source 1..24: mol_type = other DNA
aaccatgcacagaatccagattta

SEQ ID NO: 133 - DNA, 20 bp, synthetic construct
  misc_feature 1..20: note = KDM4C forward primer
  source 1..20: mol_type = other DNA
agccacccttggttggtttt

SEQ ID NO: 134 - DNA, 20 bp, synthetic construct
  misc_feature 1..20: note = KDM4C reverse primer
  source 1..20: mol_type = other DNA
ttctctccagacactgccct

SEQ ID NO: 135 - DNA, 26 bp, synthetic construct
  misc_feature 1..26: note = NF1 forward primer
  source 1..26: mol_type = other DNA
gccattattgacaagaagtctagggc

SEQ ID NO: 136 - DNA, 26 bp, synthetic construct
  misc_feature 1..26: note = NF1 reverse primer
  source 1..26: mol_type = other DNA
gcaaattccccaaaacacagtaaccc

SEQ ID NO: 137 - DNA, 25 bp, synthetic construct
  misc_feature 1..25: note = NF2 forward primer
  source 1..25: mol_type = other DNA
gggacctgctgaaacttgtcacatg

SEQ ID NO: 138 - DNA, 27 bp, synthetic construct
  misc_feature 1..27: note = NF2 reverse primer
  source 1..27: mol_type = other DNA
ccagtctgggcatgcataatgaaatcc

SEQ ID NO: 139 - DNA, 23 bp, synthetic construct
  misc_feature 1..23: note = PRMT2 forward primer
  source 1..23: mol_type = other DNA
attgccttaagtcgacacctgat

SEQ ID NO: 140 - DNA, 20 bp, synthetic construct
  misc_feature 1..20: note = PRMT2 reverse primer
  source 1..20: mol_type = other DNA
caccttacaggcactgcgtt

SEQ ID NO: 141 - DNA, 22 bp, synthetic construct
  misc_feature 1..22: note = PRMT6 forward primer
  source 1..22: mol_type = other DNA
gactgtagagttgccggaacag

SEQ ID NO: 142 - DNA, 22 bp, synthetic construct
  misc_feature 1..22: note = PRMT6 reverse primer
  source 1..22: mol_type = other DNA
ctccctccctagaggctatgag

SEQ ID NO: 143 - DNA, 23 bp, synthetic construct
  misc_feature 1..23: note = VEGFA site 3 forward primer
  source 1..23: mol_type = other DNA
tgccagactccacagtgcatacg

SEQ ID NO: 144 - DNA, 21 bp, synthetic construct
  misc_feature 1..21: note = VEGFA site 3 reverse primer
  source 1..21: mol_type = other DNA
agtgaggttacgtgcggacag

SEQ ID NO: 145 - DNA, 20 bp, synthetic construct
  misc_feature 1..20: note = VEGFA site 3 OFF1 forward primer
  source 1..20: mol_type = other DNA
atgcggtttcttccgggatt

SEQ ID NO: 146 - DNA, 20 bp, synthetic construct
  misc_feature 1..20: note = VEGFA site 3 OFF1 reverse primer
  source 1..20: mol_type = other DNA
gagaggatcgcagtccgaag

SEQ ID NO: 147 - DNA, 23 bp, synthetic construct
  misc_feature 1..23: note = VEGFA site 3 OFF2 forward primer
  source 1..23: mol_type = other DNA
gcttgcagcagaacacatgttgg

SEQ ID NO: 148 - DNA, 20 bp, synthetic construct
  misc_feature 1..20: note = VEGFA site 3 OFF2 reverse primer
  source 1..20: mol_type = other DNA
gttgcctggggatggggtat

SEQ ID NO: 149 - DNA, 22 bp, synthetic construct
  misc_feature 1..22: note = VEGFA site 3 OFF3 forward primer
  source 1..22: mol_type = other DNA
acagtgaggtgcggtctttggg

SEQ ID NO: 150 - DNA, 25 bp, synthetic construct
  misc_feature 1..25: note = VEGFA site 3 OFF3 reverse primer
  source 1..25: mol_type = other DNA
gcacctaattgatgcagtttggctc

SEQ ID NO: 151 - DNA, 24 bp, synthetic construct
  misc_feature 1..24: note = VEGFA site 3 OFF4 forward primer
  source 1..24: mol_type = other DNA
ttagctcccttgtgctgatgagac

SEQ ID NO: 152 - DNA, 24 bp, synthetic construct
  misc_feature 1..24: note = VEGFA site 3 OFF4 reverse primer
  source 1..24: mol_type = other DNA
gagatgcctgatgccgatgtaacc

SEQ ID NO: 153 - DNA, 23 bp, synthetic construct
  misc_feature 1..23: note = VEGFA site 3 OFF5 forward primer
  source 1..23: mol_type = other DNA
tctcaccacctggctcccatttc

SEQ ID NO: 154 - DNA, 20 bp, synthetic construct
  misc_feature 1..20: note = VEGFA site 3 OFF5 reverse primer
  source 1..20: mol_type = other DNA
ccaatccaggatgattccgc

SEQ ID NO: 155 - DNA, 20 bp, synthetic construct
  misc_feature 1..20: note = VEGFA site 3 OFF6 forward primer
  source 1..20: mol_type = other DNA
acagagtagctgacccacct

SEQ ID NO: 156 - DNA, 20 bp, synthetic construct
  misc_feature 1..20: note = VEGFA site 3 OFF6 reverse primer
  source 1..20: mol_type = other DNA
gctgccgtccgaacccaaga

SEQ ID NO: 157 - DNA, 23 bp, synthetic construct
  misc_feature 1..23: note = VEGFA site 3 OFF7 forward primer
  source 1..23: mol_type = other DNA
ggaggctgacagtacttcatggt

SEQ ID NO: 158 - DNA, 23 bp, synthetic construct
  misc_feature 1..23: note = VEGFA site 3 OFF7 reverse primer
  source 1..23: mol_type = other DNA
cgggactttcaccaggtccagag

SEQ ID NO: 159 - DNA, 20 bp, synthetic construct
  misc_feature 1..20: note = FANCF site 6 forward primer
  source 1..20: mol_type = other DNA
cagcatgtgcaccgcagacc

SEQ ID NO: 160 - DNA, 21 bp, synthetic construct
  misc_feature 1..21: note = FANCF site 6 reverse primer
  source 1..21: mol_type = other DNA
tcatctcgcacgtggttccgg

SEQ ID NO: 161 - DNA, 21 bp, synthetic construct
  misc_feature 1..21: note = EMX1 site 3 forward primer
  source 1..21: mol_type = other DNA
tgcttgtccctctgtcaatgg

SEQ ID NO: 162 - DNA, 20 bp, synthetic construct
  misc_feature 1..20: note = EMX1 site 3 reverse primer
  source 1..20: mol_type = other DNA
ttaggccctgtgggagatca

SEQ ID NO: 163 - DNA, 20 bp, synthetic construct
  misc_feature 1..20: note = CXCR4 forward primer
  source 1..20: mol_type = other DNA
ggagtggcctctttgtgtgt

SEQ ID NO: 164 - DNA, 20 bp, synthetic construct
  misc_feature 1..20: note = CXCR4 reverse primer
  source 1..20: mol_type = other DNA
atctgcctcactgacgttgg

SEQ ID NO: 165 - DNA, 20 bp, synthetic construct
  misc_feature 1..20: note = PD1 forward primer
  source 1..20: mol_type = other DNA
cgggatatggaaagaggcca

SEQ ID NO: 166 - DNA, 20 bp, synthetic construct
  misc_feature 1..20: note = PD1 reverse primer
  source 1..20: mol_type = other DNA
aagccaaggttagtcccaca

SEQ ID NO: 167 - DNA, 24 bp, synthetic construct
  misc_feature 1..24: note = EMX1 site 2 forward primer
  source 1..24: mol_type = other DNA
cctcctagttatgaaaccatgccc

SEQ ID NO: 168 - DNA, 20 bp, synthetic construct
  misc_feature 1..20: note = EMX1 site 2 reverse primer
  source 1..20: mol_type = other DNA
agggagattggagacacgga

SEQ ID NO: 169 - DNA, 21 bp, synthetic construct
  misc_feature 1..21: note = FANCF site 3 forward primer
  source 1..21: mol_type = other DNA
cggtaggatgccctacatctg

SEQ ID NO: 170 - DNA, 21 bp, synthetic construct
  misc_feature 1..21: note = FANCF site 3 reverse primer
  source 1..21: mol_type = other DNA
agtcctcctggagatttgggt

SEQ ID NO: 171 - DNA, 20 bp, synthetic construct
  misc_feature 1..20: note = ZSCAN2 forward primer
  source 1..20: mol_type = other DNA
agtgtggggtgtgtgggaag

SEQ ID NO: 172 - DNA, 20 bp, synthetic construct
  misc_feature 1..20: note = ZSCAN2 reverse primer
  source 1..20: mol_type = other DNA
gcaaggggaagactctggca

SEQ ID NO: 173 - DNA, 20 bp, synthetic construct
  misc_feature 1..20: note = FANCF site 1 forward primer
  source 1..20: mol_type = other DNA
cagaattcagcatagcgcct

SEQ ID NO: 174 - DNA, 20 bp, synthetic construct
  misc_feature 1..20: note = FANCF site 1 reverse primer
  source 1..20: mol_type = other DNA
ctgcaccaggtggtaacgag

SEQ ID NO: 175 - DNA, 20 bp, synthetic construct
  misc_feature 1..20: note = RUNX site 1 forward primer
  source 1..20: mol_type = other DNA
caaaccacagggtttcgcag

SEQ ID NO: 176 - DNA, 20 bp, synthetic construct
  misc_feature 1..20: note = RUNX site 1 reverse primer
  source 1..20: mol_type = other DNA
actcagacacaggcattccg

SEQ ID NO: 177 - DNA, 20 bp, synthetic construct
  misc_feature 1..20: note = EMX1sg1 forward primer
  source 1..20: mol_type = other DNA
aggagctaggatgcacagca

SEQ ID NO: 178 - DNA, 20 bp, synthetic construct
  misc_feature 1..20: note = EMX1sg1 reverse primer
  source 1..20: mol_type = other DNA
gaacgcgtttgctctaccag

SEQ ID NO: 179 - DNA, 22 bp, synthetic construct
  misc_feature 1..22: note = DMD forward primer
  source 1..22: mol_type = other DNA
gcttattcttccccagggtgat

SEQ ID NO: 180 - DNA, 20 bp, synthetic construct
  misc_feature 1..20: note = DMD reverse primer
  source 1..20: mol_type = other DNA
agttcctgctcttcgctaca

SEQ ID NO: 181 - DNA, 20 bp, synthetic construct
  misc_feature 1..20: note = AAVS forward primer
  source 1..20: mol_type = other DNA
ggctggctactggccttatc

SEQ ID NO: 182 - DNA, 20 bp, synthetic construct
  misc_feature 1..20: note = AAVS reverse primer
  source 1..20: mol_type = other DNA
ctcctgtggattcgggtcac

SEQ ID NO: 183 - DNA, 21 bp, synthetic construct
  misc_feature 1..21: note = HPRT forward primer
  source 1..21: mol_type = other DNA
ggcaaaggatgtgttacgtgg

SEQ ID NO: 184 - DNA, 21 bp, synthetic construct
  misc_feature 1..21: note = HPRT reverse primer
  source 1..21: mol_type = other DNA
cgccaatactctagctctcca

SEQ ID NO: 185 - DNA, 21 bp, synthetic construct
  misc_feature 1..21: note = HPRT38087 forward primer
  source 1..21: mol_type = other DNA
gtgatgctcacctctcccaca

SEQ ID NO: 186 - DNA, 21 bp, synthetic construct
  misc_feature 1..21: note = HPRT38087 reverse primer
  source 1..21: mol_type = other DNA
acaagaagtgtcaccctagcc

SEQ ID NO: 187 - DNA, 20 bp, synthetic construct
  misc_feature 1..20: note = FANCF site 2 forward primer
  source 1..20: mol_type = other DNA
cagcatgtgcaccgcagacc

SEQ ID NO: 188 - DNA, 21 bp, synthetic construct
  misc_feature 1..21: note = FANCF site 2 reverse primer
  source 1..21: mol_type = other DNA
tcatctcgcacgtggttccgg

SEQ ID NO: 189 - DNA, 20 bp, synthetic construct
  misc_feature 1..20: note = FANCF site 1 forward primer
  source 1..20: mol_type = other DNA
cagaattcagcatagcgcct

SEQ ID NO: 190 - DNA, 20 bp, synthetic construct
  misc_feature 1..20: note = FANCF site 1 reverse primer
  source 1..20: mol_type = other DNA
ctgcaccaggtggtaacgag

SEQ ID NO: 191 - DNA, 48 bp, synthetic construct
  misc_feature 1..48: note = OFF_GSP1_- primer
  source 1..48: mol_type = other DNA
ggatctcgacgctctccctgtttaattgagttgtcatatgttaataac

SEQ ID NO: 192 - DNA, 41 bp, synthetic construct
  misc_feature 1..41: note = OFF_GSP1_+ primer
  source 1..41: mol_type = other DNA
ggatctcgacgctctccctataccgttattaacatatgaca

SEQ ID NO: 193 - DNA, 45 bp, synthetic construct
  misc_feature 1..45: note = OFF_GSP2_- primer
  source 1..45: mol_type = other DNA
cctctctatgggcagtcggtgatacatatgacaactcaattaaac

SEQ ID NO: 194 - DNA, 50 bp, synthetic construct
  misc_feature 1..50: note = OFF_GSP2_+ primer
  source 1..50: mol_type = other DNA
cctctctatgggcagtcggtgatttgagttgtcatatgttaataacggta

SEQ ID NO: 195 - DNA, 58 bp, synthetic construct
  misc_feature 1..58: note = P558 primer
  source 1..58: mol_type = other DNA
aatgatacggcgaccaccgagatctacactctttccctacacgacgctcttccgatct

SEQ ID NO: 196 - DNA, 65 bp, synthetic construct
  misc_feature 1..65: note = P701 primer
  source 1..65: mol_type = other DNA
caagcagaagacggcatacgagattcgccttagtgactggagtcctctctatgggcagtcggtga

SEQ ID NO: 197 - DNA, 65 bp, synthetic construct
  misc_feature 1..65: note = P702 primer
  source 1..65: mol_type = other DNA
caagcagaagacggcatacgagatctagtacggtgactggagtcctctctatgggcagtcggtga

SEQ ID NO: 198 - DNA, 65 bp, synthetic construct
  misc_feature 1..65: note = P703 primer
  source 1..65: mol_type = other DNA
caagcagaagacggcatacgagatttctgcctgtgactggagtcctctctatgggcagtcggtga

SEQ ID NO: 199 - DNA, 65 bp, synthetic construct
  misc_feature 1..65: note = P704 primer
  source 1..65: mol_type = other DNA
caagcagaagacggcatacgagatgctcaggagtgactggagtcctctctatgggcagtcggtga

SEQ ID NO: 200 - DNA, 65 bp, synthetic construct
  misc_feature 1..65: note = P705 primer
  source 1..65: mol_type = other DNA
caagcagaagacggcatacgagataggagtccgtgactggagtcctctctatgggcagtcggtga

SEQ ID NO: 201 - DNA, 65 bp, synthetic construct
  misc_feature 1..65: note = P706 primer
  source 1..65: mol_type = other DNA
caagcagaagacggcatacgagatcatgcctagtgactggagtcctctctatgggcagtcggtga

SEQ ID NO: 202 - DNA, 65 bp, synthetic construct
  misc_feature 1..65: note = P707 primer
  source 1..65: mol_type = other DNA
caagcagaagacggcatacgagatgtagagaggtgactggagtcctctctatgggcagtcggtga

SEQ ID NO: 203 - DNA, 65 bp, synthetic construct
  misc_feature 1..65: note = P708 primer
  source 1..65: mol_type = other DNA
caagcagaagacggcatacgagatcctctctggtgactggagtcctctctatgggcagtcggtga

SEQ ID NO: 204 - DNA, 65 bp, synthetic construct
  misc_feature 1..65: note = P709 primer
  source 1..65: mol_type = other DNA
caagcagaagacggcatacgagatagcgtagcgtgactggagtcctctctatgggcagtcggtga

SEQ ID NO: 205 - DNA, 65 bp, synthetic construct
  misc_feature 1..65: note = P710 primer
  source 1..65: mol_type = other DNA
caagcagaagacggcatacgagatcagcctcggtgactggagtcctctctatgggcagtcggtga

SEQ ID NO: 206 - DNA, 65 bp, synthetic construct
  misc_feature 1..65: note = P711 primer
  source 1..65: mol_type = other DNA
caagcagaagacggcatacgagattgcctcttgtgactggagtcctctctatgggcagtcggtga

SEQ ID NO: 207 - DNA, 65 bp, synthetic construct
  misc_feature 1..65: note = P712 primer
  source 1..65: mol_type = other DNA
caagcagaagacggcatacgagattcctctacgtgactggagtcctctctatgggcagtcggtga

SEQ ID NO: 208 - DNA, 65 bp, synthetic construct
  misc_feature 1..65: note = P713 primer
  source 1..65: mol_type = other DNA
caagcagaagacggcatacgagataacttcacgtgactggagtcctctctatgggcagtcggtga

SEQ ID NO: 209 - DNA, 65 bp, synthetic construct
  misc_feature 1..65: note = P714 primer
  source 1..65: mol_type = other DNA
caagcagaagacggcatacgagattggagagggtgactggagtcctctctatgggcagtcggtga

SEQ ID NO: 210 - DNA, 65 bp, synthetic construct
  misc_feature 1..65: note = P715 primer
  source 1..65: mol_type = other DNA
caagcagaagacggcatacgagatacgcatcggtgactggagtcctctctatgggcagtcggtga

SEQ ID NO: 211 - DNA, 65 bp, synthetic construct
  misc_feature 1..65: note = P716 primer
  source 1..65: mol_type = other DNA
caagcagaagacggcatacgagatgtaccgttgtgactggagtcctctctatgggcagtcggtga

SEQ ID NO: 212 - DNA, 65 bp, synthetic construct
  misc_feature 1..65: note = P717 primer
  source 1..65: mol_type = other DNA
caagcagaagacggcatacgagattacagttagtgactggagtcctctctatgggcagtcggtga

SEQ ID NO: 213 - DNA, 65 bp, synthetic construct
  misc_feature 1..65: note = P718 primer
  source 1..65: mol_type = other DNA
caagcagaagacggcatacgagataatcaactgtgactggagtcctctctatgggcagtcggtga

SEQ ID NO: 214 - DNA, 65 bp, synthetic construct
  misc_feature 1..65: note = P719 primer
  source 1..65: mol_type = other DNA
caagcagaagacggcatacgagatgtacctaggtgactggagtcctctctatgggcagtcggtga

SEQ ID NO: 215 - DNA, 65 bp, synthetic construct
  misc_feature 1..65: note = P720 primer
  source 1..65: mol_type = other DNA
caagcagaagacggcatacgagatctggaacagtgactggagtcctctctatgggcagtcggtga

SEQ ID NO: 216 - DNA, 65 bp, synthetic construct
  misc_feature 1..65: note = P721 primer
  source 1..65: mol_type = other DNA
caagcagaagacggcatacgagatggtgactagtgactggagtcctctctatgggcagtcggtga

SEQ ID NO: 217 - DNA, 65 bp, synthetic construct
  misc_feature 1..65: note = P722 primer
  source 1..65: mol_type = other DNA
caagcagaagacggcatacgagatgtgcaaccgtgactggagtcctctctatgggcagtcggtga

SEQ ID NO: 218 - DNA, 65 bp, synthetic construct
  misc_feature 1..65: note = P723 primer
  source 1..65: mol_type = other DNA
caagcagaagacggcatacgagatgcctgtctgtgactggagtcctctctatgggcagtcggtga

SEQ ID NO: 219 - DNA, 65 bp, synthetic construct
  misc_feature 1..65: note = P724 primer
  source 1..65: mol_type = other DNA
caagcagaagacggcatacgagatactgatgggtgactggagtcctctctatgggcagtcggtga

SEQ ID NO: 220 - DNA, 65 bp, synthetic construct
  misc_feature 1..65: note = P725 primer
  source 1..65: mol_type = other DNA
caagcagaagacggcatacgagatatgctaacgtgactggagtcctctctatgggcagtcggtga

SEQ ID NO: 221 - DNA, 65 bp, synthetic construct
  misc_feature 1..65: note = P726 primer
  source 1..65: mol_type = other DNA
caagcagaagacggcatacgagatcactgagtgtgactggagtcctctctatgggcagtcggtga

SEQ ID NO: 222 - DNA, 65 bp, synthetic construct
  misc_feature 1..65: note = P727 primer
  source 1..65: mol_type = other DNA
caagcagaagacggcatacgagattaggccatgtgactggagtcctctctatgggcagtcggtga

SEQ ID NO: 223 - DNA, 65 bp, synthetic construct
  misc_feature 1..65: note = P728 primer
  source 1..65: mol_type = other DNA
caagcagaagacggcatacgagatcagcagtcgtgactggagtcctctctatgggcagtcggtga

SEQ ID NO: 224 - DNA, 65 bp, synthetic construct
  misc_feature 1..65: note = P729 primer
  source 1..65: mol_type = other DNA
caagcagaagacggcatacgagatttctgagagtgactggagtcctctctatgggcagtcggtga

SEQ ID NO: 225 - DNA, 65 bp, synthetic construct
  misc_feature 1..65: note = P730 primer
  source 1..65: mol_type = other DNA
caagcagaagacggcatacgagatggacgttagtgactggagtcctctctatgggcagtcggtga

SEQ ID NO: 226 - DNA, 65 bp, synthetic construct
  misc_feature 1..65: note = P731 primer
  source 1..65: mol_type = other DNA
caagcagaagacggcatacgagatgtgtaggtgtgactggagtcctctctatgggcagtcggtga

SEQ ID NO: 227 - DNA, 65 bp, synthetic construct
  misc_feature 1..65: note = P732 primer
  source 1..65: mol_type = other DNA
caagcagaagacggcatacgagatcatctcaggtgactggagtcctctctatgggcagtcggtga

SEQ ID NO: 228 - DNA, 65 bp, synthetic construct
  misc_feature 1..65: note = P733 primer
  source 1..65: mol_type = other DNA
caagcagaagacggcatacgagatgcatagcagtgactggagtcctctctatgggcagtcggtga

SEQ ID NO: 229 - DNA, 65 bp, synthetic construct
  misc_feature 1..65: note = P734 primer
  source 1..65: mol_type = other DNA
caagcagaagacggcatacgagatcagtgcacgtgactggagtcctctctatgggcagtcggtga

SEQ ID NO: 230 - DNA, 65 bp, synthetic construct
  misc_feature 1..65: note = P735 primer
  source 1..65: mol_type = other DNA
caagcagaagacggcatacgagatttcggcatgtgactggagtcctctctatgggcagtcggtga

SEQ ID NO: 231 - DNA, 65 bp, synthetic construct
  misc_feature 1..65: note = P736 primer
  source 1..65: mol_type = other DNA
caagcagaagacggcatacgagatcaacaggtgtgactggagtcctctctatgggcagtcggtga

SEQ ID NO: 232 - DNA, 65 bp, synthetic construct; identical to SEQ ID NO: 231
  misc_feature 1..65: note = P736 primer
  source 1..65: mol_type = other DNA

SEQ ID NO: 233 - DNA, 65 bp, synthetic construct
  misc_feature 1..65: note = P737 primer
  source 1..65: mol_type = other DNA
caagcagaagacggcatacgagataacactcggtgactggagtcctctctatgggcagtcggtga

SEQ ID NO: 234 - DNA, 65 bp, synthetic construct
  misc_feature 1..65: note = P738 primer
  source 1..65: mol_type = other DNA
caagcagaagacggcatacgagatgtcctgacgtgactggagtcctctctatgggcagtcggtga

SEQ ID NO: 235 - DNA, 65 bp, synthetic construct
  misc_feature 1..65: note = P739 primer
  source 1..65: mol_type = other DNA
caagcagaagacggcatacgagatgacgtagagtgactggagtcctctctatgggcagtcggtga

SEQ ID NO: 236 - DNA, 65 bp, synthetic construct
  misc_feature 1..65: note = P740 primer
  source 1..65: mol_type = other DNA
caagcagaagacggcatacgagatgattggcagtgactggagtcctctctatgggcagtcggtga

SEQ ID NO: 237 - DNA, 65 bp, synthetic construct
  misc_feature 1..65: note = P741 primer
  source 1..65: mol_type = other DNA
caagcagaagacggcatacgagatgccacgacgtgactggagtcctctctatgggcagtcggtga

SEQ ID NO: 238 - DNA, 65 bp, synthetic construct
  misc_feature 1..65: note = P742 primer
  source 1..65: mol_type = other DNA
caagcagaagacggcatacgagatttgttacggtgactggagtcctctctatgggcagtcggtga

SEQ ID NO: 239 - DNA, 65 bp, synthetic construct
  misc_feature 1..65: note = P743 primer
  source 1..65: mol_type = other DNA
caagcagaagacggcatacgagatacgacctagtgactggagtcctctctatgggcagtcggtga

SEQ ID NO: 240 - DNA, 65 bp, synthetic construct
  misc_feature 1..65: note = P744 primer
  source 1..65: mol_type = other DNA
caagcagaagacggcatacgagattgataatggtgactggagtcctctctatgggcagtcggtga

SEQ ID NO: 241 - DNA, 65 bp, synthetic construct
  misc_feature 1..65: note = P745 primer
  source 1..65: mol_type = other DNA
caagcagaagacggcatacgagatggttccatgtgactggagtcctctctatgggcagtcggtga

SEQ ID NO: 242 - DNA, 65 bp, synthetic construct
  misc_feature 1..65: note = P746 primer
  source 1..65: mol_type = other DNA
caagcagaagacggcatacgagatccagtatcgtgactggagtcctctctatgggcagtcggtga

SEQ ID NO: 243 - DNA, 65 bp, synthetic construct
  misc_feature 1..65: note = P747 primer
  source 1..65: mol_type = other DNA
caagcagaagacggcatacgagatgtccagctgtgactggagtcctctctatgggcagtcggtga

SEQ ID NO: 244 - DNA, 65 bp, synthetic construct
  misc_feature 1..65: note = P748 primer
  source 1..65: mol_type = other DNA
caagcagaagacggcatacgagattaaccttcgtgactggagtcctctctatgggcagtcggtga

SEQ ID NO: 245 - DNA, 34 bp, synthetic construct
  misc_feature 1..34: note = Custom sequencing primer Index1
  source 1..34: mol_type = other DNA
atcaccgactgcccatagagaggactccagtcac

SEQ ID NO: 246 - DNA, 34 bp, synthetic construct
  misc_feature 1..34: note = Custom sequencing primer Read2
  source 1..34: mol_type = other DNA
gtgactggagtcctctctatgggcagtcggtgat

SEQ ID NO: 247 - DNA, 20 bp, synthetic construct
  misc_feature 1..20: note = VEGFA OFF1
  source 1..20: mol_type = other DNA
agtgagtgagtgtgtgtgtg

SEQ ID NO: 248 - DNA, 20 bp, synthetic construct
  misc_feature 1..20: note = VEGFA OFF2
  source 1..20: mol_type = other DNA
tgtgggtgagtgtgtgcgtg

SEQ ID NO: 249 - DNA, 20 bp, synthetic construct
  misc_feature 1..20: note = VEGFA OFF3
  source 1..20: mol_type = other DNA
agagagtgagtgtgtgcatg

SEQ ID NO: 250 - DNA, 20 bp, synthetic construct
  misc_feature 1..20: note = VEGFA OFF4
  source 1..20: mol_type = other DNA
agtgtgtgagtgtgtgcgtg

SEQ ID NO: 251 - DNA, 20 bp, synthetic construct
  misc_feature 1..20: note = VEGFA OFF5
  source 1..20: mol_type = other DNA
gctgagtgagtgtatgcgtg

SEQ ID NO: 252 - DNA, 20 bp, synthetic construct
  misc_feature 1..20: note = VEGFA OFF6
  source 1..20: mol_type = other DNA
ggtgagtgagtgcgtgcggg

SEQ ID NO: 253 - DNA, 22 bp, synthetic construct
  misc_feature 1..22: note = VEGFA OFF7
  source 1..22: mol_type = other DNA
gttgagtgaatgtgtgtgcgtg

SEQ ID NO: 254 - DNA, 20 bp, synthetic construct
  misc_feature 1..20: note = DNMT1 OFF1
  source 1..20: mol_type = other DNA
ggagggagggaaacagcccc

SEQ ID NO: 255 - protein, 524 aa, Streptococcus pyogenes
DKSGASEEATCSNAKDSHEKHEHNVVAEKKTDVIGDLNPDSDDLIQLQTNQLENPINASRVDAKALARLNAQLGKNGNLASLTPNSNDADKLNQQANSTDRNSEIKDEHQTLALQQPEKKFQNGASEPETELANLYGHEDKREKNSRTKSETTKGAQSEKNNYTVTGMKPALSGEQKAVDLTNVQKEDYFKKECSSDRTGKDNEEDDLEEEKKANDKQKDRRQGKKSFANDSAQSQGHSHEQANAHKENQKQKREMREGESQLKEHPVNTQVDQENRDSDRDKNEKMNRQNAQDSLAQSMTKYDNDLEKDQFNTKKSKVDVRMIAKSEQEIGKAYFTEITLANGEIRKRPLIETNGTGIVDKGDFATMVTGFSKESLPRNSDKLIARKDWPKDSTVASVKVEKSKSVKELSSKNPDEAKERKDLLENSRAGELKGNELALPSKYNFLYLASHEKLKGSPEDNEQQLEQKHYLDEQSESKVLDALDLSANKHRDKPREQAENIHFTLTNLAFDTTDTTKEDSQGD

SEQ ID NO: 256 - protein, 520 aa, Streptococcus dysgalactiae
DKSFSASEEATRSSSKDSHEKHEHNVVAEKKTDIGDLNPDSDDLIQLQTNQLENPINASRVDAKALARLNAQLGRNGNLASLTPNSNDADKLNQQANSDRNSEIKDEHQTLALQQPEKKFQNGASEPETELANLGHEDKREKNSRTKSETTKGAQSEKNNYTVTGMKPALSGEQKAVDLTNVQKEDYFKKECSSDRAGKDNEEDDLEEEKKANDKQKRRQGKKSFANDSAQSQGHSHEQANAHKENQKQKREMREGESQLKEHPVNTQVDQENRDSDRDKNEKMNRQNAQDSLAQSMTKYDNDLEKDQFNTKKSKVDVRMIAKSEQEIGKARFTEITLANGEIRKRPLIETNETGIVDKGDFATMVTGLTNESYAGSFDKLISRHRFSSGSTVTSVKSKVQDKVKTGKEILVKNPKEDGNQIDKCFENTVMANNSRGDLQEMFPAKLVTHKIESSKELEEALDYNDLYQSYERASLDVEKISKELSNIESYSSECSVNLTLTASDLGTTPGPQSSSSQGD

SEQ ID NO: 257 - protein, 527 aa, Streptococcus equi
KPVTTASDEGTPRKTEAKDGQYLEGNHNAVAKKEVNPQIGTLSSKNNQSDHLDTNLLEQRLLTEGINAKELAAKLNSLIGQKTGNIASLTPNANGSKDVKLAASQQANSDESEIKREHKVTTLDQPEKQLKNQVSEPASPLLEHEVKRKESHSRKKFGAREEAQIEKNLNTTATGMTRPQLSADQQAVDLTNVQKENYFKKECSTDSAGQDNPDQKDLKSKDQAHKVNKEHRQGKKAFAHSEIEAIKTEYSKDGNASYLQQAQIKARQMKETAKSNLKEHPVNSQRDDDYSSNNQGALNEARMGQSRAGAKQDTQVAQLQSTEFDHNRKKDGHKGKQAPKNSFERQKQTLKDQESLHVNSDGEINANHLPINIVTGFYKESLSGNSDKLIPRNNWTRDSTVASIKMEKAVKPVKEVIAENPVEAREQEHLLENRASELKGNELFLPVDYTFLYLAAHELTGSSEDVLRKYERLHYDQMNDAEHLSSLENHTHNNSDLPNERAENINFTFVALAFDATDTTKENSQEN

SEQ ID NO: 258 - protein, 514 aa, Streptococcus mutans
KPASHASNEDRLSEGKDSHTDNFDSHNKADAQKHTEIGELNAETDQLADFGVDRTDSHLSEITVDASSLERLKNNYKKNTGNLASLQPNTNKSDKFVQNSKYSGTVSQNEQMAQQFQKSDKNSVDKTNAGNSGYFDQRAEAQEKKSDKSADKTKESVEANLNQKTKTQGKTAFDANMQEFDGVYKDKMDFLEKEFDERITKENKAAYGRDNSKKDLERKKNSDLTKEQKEEHRNERKIDNSNDAEAIETDNNQSDAHQENFNQRRQQLGTDSEFSQLKEHPVNSQEEDYQANKEDKRMSSKSAQDTDARETETDNNKQNNEDKGVQPHHGHENKAAKFKDESLHVNSDGEINANHLPINIVTGFYKESLSGNSDKLIPRNNWTRDSTVASIKMEKAVKPVKEVIAENPVEAREQEHLLENRASELKGNELFLPVDYTFLYLAAHELTGSSEDVLRKYERLHYDQMNDAEHLSSLENHTHNNSDLPNERAENINFTFVALAFDATDTTKENSQEN

SEQ ID NO: 259 - protein, 520 aa, Streptococcus oralis
MNNPSFAETEDRRTESKSNHPRGSYTEKEKNHKEFYESFDIKNDQINEFSIDNTGSSLNGQNAQVEAFDARRKLFDSTSEFKINQADKHDEKPFNQDVKYGTPSEENQKATQFNNPEKDSQDKTTANSAYFDQNGEHQKEKNRDTNSQARKAREDNLETAIAGLDYQLDSGQKQVTQEKEDIQYLHTDGGKKQASKDDSKANHERQTQASEKATCQGDIDEIHDGIQVKTDDKQQEPHEESARKKQQYRDANPEDSNILKHPTDNIQEANQSCADKDNLQRAQQDSENDRVQATEVTKDKDSNNRDKKKQKDLKYISRTKDPKEVEKEYFEEVHYADGTIVKRENIEYSKTGIANKEDFATLETVQNGGLFDNNVSKKVVDASKLTPISGLSPEARTIASIDIEKAKRIKEVQKKANPAEECKNNPNLFNNQSIELELIPYHFTAQRINKISEPIKQETQSEKTAISLSKQKPVESLQQAFDQSDKDYQSEFSLKLISFTLGVESQSNVQVSSCFNSKED

SEQ ID NO: 260 - protein, 545 aa, Streptococcus mitis
MNNNNSFAETEDRRSPSKSSHPRGSYTAKEKNQKEYESFDIKNDQINEFSIDNTGSSLSGQNAQVEAFDARRKLFDSTSEFKINQAEKHDEKPFNQGAKYGTPSEENQKAAQFQNNQEKDSQDNKTTANSFSYFDQNGEHQKKKNGDTNSQARQASEDNLETAIAGLDYQLDSGQKQVNQEKEDTQYLHNDGGKKQASKDADAEATNHEKQAQDSEKAICKGKIDYSNDGIQVRTNDKQHEPHTESARKKQQYRDANPGDSNILKYPTDNIQEPNQSADKDNLQRAQQDSENDRVQATEVTKDKNNNNKDKKKQKDLKYISRSKDPKDVEKEYFEEVHYADGTIVKRENIEYSKTGIANKEDFATLITHLDRGKPRGLFNSNPSPPSEDSKENLVPIQGLPRAGISNSAKIIEAKQQKTVLEFQINKNKENLEIKLSTTFPDTRILSTNKRGEIHELVSEKYTTKNINKTLEPELEEKRNDAKESLDNDGLKGERQAIDWETVDEKCFFGPRNSKNAGFELTSQSASDELGVKPYDYPSSNSKED

SEQ ID NO: 261 - protein, 507 aa, Streptococcus parasanguis
KPANESAANADRLAANKESHPRGSYTEKEKQYIKEVYDSFDIKNDQINEFTILDNTESSLSKGNAQVEEFDARRKLFDSTSEFKINQADKHDEKPFSQVVKYAGKPGEDNQNSAQFRNPEKASDDKTTGNSAYFEQNGEKKEQNSDSNSEARKSSEDHLETTIAGMDYQLDSGQKQVNQEKEDIHYLHNDGGKKHSSKDDPKEFNHVKQNQDSEKATRKSKIDYSNDGTQVETNDKQQEPHAESNKKSKQQLTSDASESNILKHPTDNIQEANQNADKDNLEMGQQDSENDRVQDAEVNKNQKSNNGDKKKQKDLKYISRTKDPKEIEKEYFDKVYYADGTIIQRGNVEYSKTGIANKKDFAIYETGFSKESLPGNSDKLIPRKTKNVQLTTDSVIASVDVEKSKTVKSIVKANPAEGQNVEENLENRAKELEMVPSYLIAKRIQKKDEPELEKQHSENNFSESQLESLEKNLIDNEQTNEEANFNLTFTAFVFGKDESVTEKSKEE

SEQ ID NO: 262 - protein, 561 aa, Streptococcus thermophilus
TPTNSSYVSIEGRLSTATDAQPRDSYNVKADEYTKIGEFNSKNDQNQDFDTNAISDLSLENSKQLEEVKDLEKRKLFGNSSEFKINQADKCNDKSHFTYDSKKYGFTNEESAKNEKEALEYNISLKTNKDNKTNDVKAFAYFEYQRDAKAKKEKNSDSIKRNEKTKESEANSLETNIASMDYQLDSKQKDVRLYDKDDIEYLHAYGGKKQSSNNDDSSAEHEKQSKENKSKSREKGNIDISHDAKKQIDEDKGNKEKSPGRKESYNQKSQQLRKSESKLKENIPAKLSKIDNNADDDRNANVASDLKRTYQKSQDSPEAQRENKKDNNATTQEDSKKPKNSFERKSEVYIKSISLADGRVIERPLIEVNETGSVNKESDLATYVENHLDRGKPKGLFNANSSPKPNSNENLVGAEYLPKAGISNSAKTIEAKTNVLEFQINRKDKNLEKDELELSDSILSTNKRGEIHQIFSQKFVKKRISNTINENRKENKKEEFYYLENENGKKGKLNSAQSWQNHSDECSFGPTGSERKGFELTSRSADELGVKPYDTPSSLKDAKEG

SEQ ID NO: 263 - protein, 577 aa, Listeria monocytogenes
KNPQDVKAQFWVREEADRNIESALANANCNYDSRNSHFTEVAKNREEVNSENIGALDTKTSDGVKQFQTNQVISNIEEGTLAKMEENTTVADLAGFKELRQLYGSTAQFSISKGNQKVDVKTDECAAIEANTYNSTTENKEDAEKSEAFLHPKQESNVAIDKTKVDTENAYFAENAEEQAKKAYKSNQSDTKAGERIKFGKVDEKTKNYQKMIDQGTNYSGQEQQFNDYQKKDEQFLRNSHISPTEDSSYAGIKQVNPLTEDKIRKEQQQSDLGAKEVRQHLMNDGLLNSNSIEESTTDKDQSADASYPQTVKKNRPYSKAEFSQLKEHPTNQERNQEHNNSTNLAGEGDPLRRVEKFQGNKDYTAATNNHQNETDNHGNNEQMAQQQDNTVQHQDWFANKAKQLAQKERIIDNGEILWDKYLETDYRIKGEFSKATKPGNSSKLIPRENWPMLDSNMAAEHAKGVFEKKIRKAKDEKSEKQRQPKVTCENRANEAQQVKGQLITHKNCEASDGKSLDESNREMGAHSEAKTLDALSNQLEQNKDNDKVAQFNMAFNAMSFEATETNLKESYAKRDG

SEQ ID NO: 264 - protein, 564 aa, Enterococcus timonesis
GDRLDVKFAFWVSEQADAMLAVEFQKAMNEKANHNEEFNHKEKAYKKETQQIGKLSTETSSETKVFDKNEASKIADNELKLDTTIDVEKLESRANNFFTKNDTDQFKINQGNKTDDDKFDTNMAGEANAYNEGQSLKGKDDKEALKFFLNNGYEEYVSFKGDGKKDNNSHTKDSTKDAYFAQVEKEGEKFQVDFNSKENHGRENSEPTITMNKEKETNKTSTDQETHNSSIEEKFKECKNKDRQKFLYNEYNLNTNNEAKAFNVSPMNDPEDFEKMKAKQASKSYEKTEVYYQQGKVMDAPGKNTNNGRKIQPYNKSNEQSKLKDYPTNKAKHDNNNSVNVKEDLNIKSRGEQHSKDTDARETEKDQTGKTATQNQDNTIQHRDSFENRAKNMTKDVTLDKGNGEILWDNSVAMDYRIRGFSNETLPGPSDKLIPRNNWPAVGSTEASSYEKGSKVVKEIGQKAENEGKTENPKVAFADRSKESQLVSKDLNEKNSDKKSESLETNNSTMFFEYDIAQITKSEQIVAENNKDSEGKDATFFNLQFTAMDFNETPSTSENYRNGD